European Patent Specification EP 3 516 044 B1, published April 16, 2025. Title: TCRS SPECIFIC FOR MINOR HISTOCOMPATIBILITY (H) ANTIGEN HA-1 AND USES THEREOF. Applicant: Fred Hutchinson Cancer Research Center Bleakley, Marie Dossa, Robson Sommermeyer, Daniel. Application PCT. The sequence listing filed with the application follows.

SEQUENCE LISTING (127 sequences)

SEQ ID NO: 1 - protein, 133 aa, Artificial Sequence
  Synthetic sequence TCR1,13 beta chain variable region with signal peptide
MGTSLLCWMALCLLGADHADTGVSQDPRHKITKRGQNVTFRCDPISEHNRLYWYRQTLGQGPEFLTYFQNEAQLEKSRLLSDRFSAERPKGSFSTLEIQRTEQGDSAMYLCASSSTGGHNEQFFGPGTRLTVL

SEQ ID NO: 2 - protein, 134 aa, Artificial Sequence
  Synthetic sequence TCR1,13 alpha chain variable region with signal peptide
METLLGVSLVILWLQLARVNSQQGEEDPQALSIQEGENATMNCSYKTSINNLQWYRQNSGRGLVHLILIRSNEREKHSGRLRVTLDTSKKSSSLLITASRAADTASYFCATKRDSGAGSYQLTFGKGTKLSVIP

SEQ ID NO: 3 - protein, 131 aa, Artificial Sequence
  Synthetic sequence TCR2,14 beta chain variable region with signal peptide
MGTSLLCWMALCLLGADHADTGVSQDPRHKITKRGQNVTFRCDPISEHNRLYWYRQTLGQGPEFLTYFQNEAQLEKSRLLSDRFSAERPKGSFSTLEIQRTEQGDSAMYLCASSLVKGEKLFGSGTQLSVL

SEQ ID NO: 4 - protein, 131 aa, Artificial Sequence
  Synthetic sequence TCR2,14 alpha chain variable region with signal peptide
METLLGLLILWLQLQWVSSKQEVTQIPAALSVPEGENLVLNCSFTDSAIYNLQWFRQDPGKGLTSLLLIQSSQREQTSGRLNASDKSSGRSTLYIAASQPGDSATYLCAVIGLGGTYKYIFGTGTRLKVLA

SEQ ID NO: 5 - protein, 132 aa, Artificial Sequence
  Synthetic sequence TCR5 beta chain variable region with signal peptide
MGTSLLCWMALCLLGADHADTGVSQDPRHKITKRGQNVTFRCDPISEHNRLYWYRQTLGQGPEFLTYFQNEAQLEKSRLLSDRFSAERPKGSFSTLEIQRTEQGDSAMYLCASSLTTLDEQYVGPGTRLTVT

SEQ ID NO: 6 - protein, 130 aa, Artificial Sequence
  Synthetic sequence TCR5 alpha chain variable region with signal peptide
METLLGVSLVILWLQLARVNSQQGEEDPQALSIQEGENATMNCSYKTSINNLQWYRQNSGRGLVHLILIRSNEREKHSGRLRVTLDTSKKSSSLLITASRAADTASYFCATNSGNTPLVFGKGTRLSVIA

SEQ ID NO: 7 - protein, 132 aa, Artificial Sequence
  Synthetic sequence TCR10 beta chain variable region with signal peptide
MGTSLLCWMALCLLGADHADTGVSQDPRHKITKRGQNVTFRCDPISEHNRLYWYRQTLGQGPEFLTYFQNEAQLEKSRLLSDRFSAERPKGSFSTLEIQRTEQGDSAMYLCASSMLTNYEQYFGPGTRLTVT

SEQ ID NO: 8 - protein, 134 aa, Artificial Sequence
  Synthetic sequence TCR10 alpha chain variable region with signal peptide
MKKHLTTFLVILWLYFYRGNGKNQVEQSPQSLIILEGKNCTLQCNYTVSPFSNLRWYKQDTGRGPVSLTIMTFSENTKSNGRYTATLDADTKQSSLHITASQLSDSASYICVVDSGGGADGLTFGKGTHLIIQP

SEQ ID NO: 9 - protein, 132 aa, Artificial Sequence
  Synthetic sequence TCR16 beta chain variable region with signal peptide
MGTSLLCWMALCLLGADHADTGVSQDPRHKITKRGQNVTFRCDPISEHNRLYWYRQTLGQGPEFLTYFQNEAQLEKSRLLSDRFSAERPKGSFSTLEIQRTEQGDSAMYLCASSLVVGNEQFFGPGTRLTVL

SEQ ID NO: 10 - protein, 131 aa, Artificial Sequence
  Synthetic sequence TCR16 alpha chain variable region with signal peptide
METLLGLLILWLQLQWVSSKQEVTQIPAALSVPEGENLVLNCSFTDSAIYNLQWFRQDPGKGLTSLLLIQSSQREQTSGRLNASLDKSSGRSTLYIAASQPGDSATYLCAVHLLNDYKLSFGAGTTVTVRA

SEQ ID NO: 11 - protein, 132 aa, Artificial Sequence
  Synthetic sequence TCR29 beta chain variable region with signal peptide
MGTSLLCWMALCLLGADHADTGVSQDPRHKITKRGQNVTFRCDPISEHNRLYWYRQTLGQGPEFLTYFQNEAQLEKSRLLSDRFSAERPKGSFSTLEIQRTEQGDSAMYLCASSLVSGNTIYFGEGSWLTVV

SEQ ID NO: 12 - protein, 134 aa, Artificial Sequence
  Synthetic sequence TCR29 alpha chain variable region with signal peptide
METLLGLLILWLQLQWVSSKQEVTQIPAALSVPEGENLVLNCSFTDSAIYNLQWFRQDPGKGLTSLLLIQSSQREQTSGRLNASLDKSSGRSTLYIAASQPGDSATYLCAVRGGTTSGTYKYIFGTGTRLKVLA

SEQ ID NO: 13 - protein, 14 aa, Artificial Sequence
  Synthetic sequence TCR1 beta chain CDR3
CASSSTGGHNEQFF

SEQ ID NO: 14 - protein, 12 aa, Artificial Sequence
  Synthetic sequence TCR2 beta chain CDR3
CASSLVKGEKLF

SEQ ID NO: 15 - protein, 13 aa, Artificial Sequence
  Synthetic sequence TCR5 beta chain CDR3
CASSLTTLDEQYV

SEQ ID NO: 16 - protein, 13 aa, Artificial Sequence
  Synthetic sequence TCR10 beta chain CDR3
CASSMLTNYEQYF

SEQ ID NO: 17 - protein, 13 aa, Artificial Sequence
  Synthetic sequence TCR16 beta chain CDR3
CASSLVVGNEQFF

SEQ ID NO: 18 - protein, 177 aa, Artificial Sequence
  Synthetic sequence TCR1,5,10,13,16 beta chain constant region (Cys modified)
EDLKNVFPPEVAVFEPSEAEISHTQKATLVCLATGFYPDHVELSWWVNGKEVHSGVCTDPQPLKEQPALNDSRYCLSSRLRVSATFWQNPRNHFRCQVQFYGLSENDEWTQDRAKPVTQIVSAEAWGRADCGFTSESYQQGVLSATILYEILLGKATLYAVLVSALVLMAMVKRKDS

SEQ ID NO: 19 - protein, 141 aa, Artificial Sequence
  Synthetic sequence TCR1,13 alpha chain constant region (Cys modified)
NIQNPDPAVYQLRDSKSSDKSVCLFTDFDSQTNVSQSKDSDVYITDKCVLDMRSMDFKSNSAVAWSNKSDFACANAFNNSIIPEDTFFPSPESSCDVKLVEKSFETDTNLNFQNLSVIGFRILLLKVAGFNLLMTLRLWSS

SEQ ID NO: 20 - protein, 201 aa, Artificial Sequence
  Synthetic sequence TCR5 alpha chain constant region (Cys modified)
NIQNPDPAVYQLRDSKSSDKSVCLFTDFDSQTNVSQSKDSDVYITDKCVLDMRSMDFKSNSAVAWSNKSDFACANAFNNSIIPEDTFFPSPESSCDVKLVEKSFETDTNLNFQNLSVIGFRILLLKVAGFNLLMTLRLWSSFACANAFNNSIIPEDTFFPSPESSCDVKLVEKSFETDTNLNFQNLSVIGFRILLLKVAGF

SEQ ID NO: 21 - protein, 81 aa, Artificial Sequence
  Synthetic sequence TCR10 alpha chain constant region (Cys modified)
YIQNPDPAVYQLRDSKSSDKSVCLFTDFDSQTNVSQSKDSDVYITDKCVLDMRSMDFKSNSAVAWSNKSDNLLMTLRLWSS

SEQ ID NO: 22 - protein, 141 aa, Artificial Sequence; identical to SEQ ID NO: 19
  Synthetic sequence TCR16 alpha chain constant region (Cys modified)

SEQ ID NO: 23 - protein, 176 aa, Artificial Sequence
  Synthetic sequence TCR2,14 beta chain constant region (Cys modified)
EDLNKVFPPEVAVFEPSEAEISHTQKATLVCLATGFFPDHVELSWWVNGKEVHSGVCTDPQPLKEQPALNDSRYCLSSRLRVSATFWQNPRNHFRCQVQFYGLSENDEWTQDRAKPVTQIVSAEAWGRADCGFTSVSYQQGVLSATILYEILLGKATLYAVLVSALVLMAMVKRKD

SEQ ID NO: 24 - protein, 141 aa, Artificial Sequence; identical to SEQ ID NO: 19
  Synthetic sequence TCR2,14 alpha chain constant region (Cys modified)

SEQ ID NO: 25 - protein, 177 aa, Artificial Sequence
  Synthetic sequence TCR29 beta chain constant region
EDLNKVFPPEVAVFEPSEAEISHTQKATLVCLATGFFPDHVELSWWVNGKEVHSGVSTDPQPLKEQPALNDSRYCLSSRLRVSATFWQNPRNHFRCQVQFYGLSENDEWTQDRAKPVTQIVSAEAWGRADCGFTSVSYQQGVLSATILYEILLGKATLYAVLVSALVLMAMVKRKDF

SEQ ID NO: 26 - protein, 141 aa, Artificial Sequence
  Synthetic sequence TCR29 alpha chain constant region
NIQNPDPAVYQLRDSKSSDKSVCLFTDFDSQTNVSQSKDSDVYITDKTVLDMRSMDFKSNSAVAWSNKSDFACANAFNNSIIPEDTFFPSPESSCDVKLVEKSFETDTNLNFQNLSVIGFRILLLKVAGFNLLMTLRLWSS

SEQ ID NO: 27 - protein, 310 aa, Artificial Sequence
  Synthetic sequence TCR1,13 beta chain (full length) (Cys modified)
MGTSLLCWMALCLLGADHADTGVSQDPRHKITKRGQNVTFRCDPISEHNRLYWYRQTLGQGPEFLTYFQNEAQLEKSRLLSDRFSAERPKGSFSTLEIQRTEQGDSAMYLCASSSTGGHNEQFFGPGTRLTVLEDLKNVFPPEVAVFEPSEAEISHTQKATLVCLATGFYPDHVELSWWVNGKEVHSGVCTDPQPLKEQPALNDSRYCLSSRLRVSATFWQNPRNHFRCQVQFYGLSENDEWTQDRAKPVTQIVSAEAWGRADCGFTSESYQQGVLSATILYEILLGKATLYAVLVSALVLMAMVKRKDS

SEQ ID NO: 28 - protein, 275 aa, Artificial Sequence
  Synthetic sequence TCR1,13 alpha chain (full length) (Cys modified) with signal peptide
METLLGVSLVILWLQLARVNSQQGEEDPQALSIQEGENATMNCSYKTSINNLQWYRQNSGRGLVHLILIRSNEREKHSGRLRVTLDTSKKSSSLLITASRAADTASYFCATKRDSGAGSYQLTFGKGTKLSVIPNIQNPDPAVYQLRDSKSSDKSVCLFTDFDSQTNVSQSKDSDVYITDKCVLDMRSMDFKSNSAVAWSNKSDFACANAFNNSIIPEDTFFPSPESSCDVKLVEKSFETDTNLNFQNLSVIGFRILLLKVAGFNLLMTLRLWSS

SEQ ID NO: 29 - protein, 308 aa, Artificial Sequence
  Synthetic sequence TCR2,14 beta chain (full length) (Cys modified) with signal peptide
MGTSLLCWMALCLLGADHADTGVSQDPRHKITKRGQNVTFRCDPISEHNRLYWYRQTLGQGPEFLTYFQNEAQLEKSRLLSDRFSAERPKGSFSTLEIQRTEQGDSAMYLCASSLVKGEKLFFGSGTQLSVLEDLNKVFPPEVAVFEPSEAEISHTQKATLVCLATGFFPDHVELSWWVNGKEVHSGVCTDPQPLKEQPALNDSRYCLSSRLRVSATFWQNPRNHFRCQVQFYGLSENDEWTQDRAKPVTQIVSAEAWGRADCGFTSVSYQQGVLSATILYEILLGKATLYAVLVSALVLMAMVKRKD

SEQ ID NO: 30 - protein, 273 aa, Artificial Sequence
  Synthetic sequence TCR2,14 alpha chain (full length) (Cys modified) with signal peptide
METLLGLLILWLQLQWVSSKQEVTQIPAALSVPEGENLVLNCSFTDSAIYNLQWFRQDPGKGLTSLLLIQSSQREQTSGRLNASLDKSSGRSTLYIAASQPGDSATYLCAVIGLGGTYKYIFGTGTRLKVLANIQNPDPAVYQLRDSKSSDKSVCLFTDFDSQTNVSQSKDSDVYITDKCVLDMRSMDFKSNSAVAWSNKSDFACANAFNNSIIPEDTFFPSPESSCDVKLVEKSFETDTNLNFQNLSVIGFRILLLKVAGFNLLMTLRLWSS

SEQ ID NO: 31 - protein, 309 aa, Artificial Sequence
  Synthetic sequence TCR5 beta chain (full length) (Cys modified) with signal peptide
MGTSLLCWMALCLLGADHADTGVSQDPRHKITKRGQNVTFRCDPISEHNRLYWYRQTLGQGPEFLTYFQNEAQLEKSRLLSDRFSAERPKGSFSTLEIQRTEQGDSAMYLCASSLTTLDEQYVGPGTRLTVTEDLKNVFPPEVAVFEPSEAEISHTQKATLVCLATGFYPDHVELSWWVNGKEVHSGVCTDPQPLKEQPALNDSRYCLSSRLRVSATFWQNPRNHFRCQVQFYGLSENDEWTQDRAKPVTQIVSAEAWGRADCGFTSESYQQGVLSATILYEILLGKATLYAVLVSALVLMAMVKRKDS

SEQ ID NO: 32 - protein, 271 aa, Artificial Sequence
  Synthetic sequence TCR5 alpha chain (full length) (Cys modified) with signal peptide
METLLGVSLVILWLQLARVNSQQGEEDPQALSIQEGENATMNCSYKTSINNLQWYRQNSGRGLVHLILIRSNEREKHSGRLRVTLDTSKKSSSLLITASRAADTASYFCATNSGNTPLVFGKGTRLSVIANIQNPDPAVYQLRDSKSSDKSVCLFTDFDSQTNVSQSKDSDVYITDKCVLDMRSMDFKSNSAVAWSNKSDFACANAFNNSIIPEDTFFPSPESSCDVKLVEKSFETDTNLNFQNLSVIGFRILLLKVAGFNLLMTLRLWSS

SEQ ID NO: 33 - protein, 309 aa, Artificial Sequence
  Synthetic sequence TCR10 beta chain (full length) (Cys modified) with signal peptide
MGTSLLCWMALCLLGADHADTGVSQDPRHKITKRGQNVTFRCDPISEHNRLYWYRQTLGQGPEFLTYFQNEAQLEKSRLLSDRFSAERPKGSFSTLEIQRTEQGDSAMYLCASSMLTNYEQYFGPGTRLTVTEDLKNVFPPEVAVFEPSEAEISHTQKATLVCLATGFYPDHVELSWWVNGKEVHSGVCTDPQPLKEQPALNDSRYCLSSRLRVSATFWQNPRNHFRCQVQFYGLSENDEWTQDRAKPVTQIVSAEAWGRADCGFTSESYQQGVLSATILYEILLGKATLYAVLVSALVLMAMVKRKDS

SEQ ID NO: 34 - protein, 275 aa, Artificial Sequence
  Synthetic sequence TCR10 alpha chain (full length) (Cys modified) with signal peptide
MKKHLTTFLVILWLYFYRGNGKNQVEQSPQSLIILEGKNCTLQCNYTVSPFSNLRWYKQDTGRGPVSLTIMTFSENTKSNGRYTATLDADTKQSSLHITASQLSDSASYICVVDSGGGADGLTFGKGTHLIIQPYIQNPDPAVYQLRDSKSSDKSVCLFTDFDSQTNVSQSKDSDVYITDKCVLDMRSMDFKSNSAVAWSNKSDFACANAFNNSIIPEDTFFPSPESSCDVKLVEKSFETDTNLNFQNLSVIGFRILLLKVAGFNLLMTLRLWSS

SEQ ID NO: 35 - protein, 308 aa, Artificial Sequence
  Synthetic sequence TCR16 beta chain (full length) (Cys modified) with signal peptide
MGTSLLCWMALCLLGADHADTGVSQDPRHKITKRGQNVTFRCDPISEHNRLYWYRQTLGQGPEFLTYFQNEAQLEKSRLLSDRFSAERPKGSFSTLEIQRTEQGDSAMYLCASSLVVGNEQFFGPGTRLTVLEDLKNVFPPEVAVFEPSEAEISHTQKATLVCLATGFYPDHVELSWWVNGKEVHSGVCTDPQPLKEQPALNDSRYCLSSRLRVSATFWQNPRNHFRCQVQFYGLSENDEWTQDRAKPVTQIVSAEAWGRADCGFTSESYQQGVLSATILYEILLGKATLYAVLVSALVLMAMVKRKD

SEQ ID NO: 36 - protein, 272 aa, Artificial Sequence
  Synthetic sequence TCR16 alpha chain (full length) (Cys modified) with signal peptide
METLLGLLILWLQLQWVSSKQEVTQIPAALSVPEGENLVLNCSFTDSAIYNLQWFRQDPGKGLTSLLLIQSSQREQTSGRLNASLDKSSGRSTLYIAASQPGDSATYLCAVHLLNDYKLSFGAGTTVTVRANIQNPDPAVYQLRDSKSSDKSVCLFTDFDSQTNVSQSKDSDVYITDKCVLDMRSMDFKSNSAVAWSNKSDFACANAFNNSIIPEDTFFPSPESSCDVKLVEKSFETDTNLNFQNLSVIGFRILLLKVAGFNLLMTLRLWSS

SEQ ID NO: 37 - protein, 309 aa, Artificial Sequence
  Synthetic sequence TCR29 beta chain (full length) (Cys modified) with signal peptide
MGTSLLCWMALCLLGADHADTGVSQDPRHKITKRGQNVTFRCDPISEHNRLYWYRQTLGQGPEFLTYFQNEAQLEKSRLLSDRFSAERPKGSFSTLEIQRTEQGDSAMYLCASSLVSGNTIYFGEGSWLTVVEDLNKVFPPEVAVFEPSEAEISHTQKATLVCLATGFFPDHVELSWWVNGKEVHSGVSTDPQPLKEQPALNDSRYCLSSRLRVSATFWQNPRNHFRCQVQFYGLSENDEWTQDRAKPVTQIVSAEAWGRADCGFTSVSYQQGVLSATILYEILLGKATLYAVLVSALVLMAMVKRKDF

SEQ ID NO: 38 - protein, 275 aa, Artificial Sequence
  Synthetic sequence TCR29 alpha chain (full length) (Cys modified) with signal peptide
METLLGLLILWLQLQWVSSKQEVTQIPAALSVPEGENLVLNCSFTDSAIYNLQWFRQDPGKGLTSLLLIQSSQREQTSGRLNASLDKSSGRSTLYIAASQPGDSATYLCAVRGGTTSGTYKYIFGTGTRLKVLANIQNPDPAVYQLRDSKSSDKSVCLFTDFDSQTNVSQSKDSDVYITDKTVLDMRSMDFKSNSAVAWSNKSDFACANAFNNSIIPEDTFFPSPESSCDVKLVEKSFETDTNLNFQNLSVIGFRILLLKVAGFNLLMTLRLWSS

SEQ ID NO: 39 - DNA, 930 bp, Artificial Sequence
  Synthetic sequence  TCR1,13 beta chain (codon optimized, Cys modified)
atgggcacctccctgctgtgttggatggccctgtgtctgctgggagccgaccatgccgatacaggggtgtcccaggacccccggcacaagattaccaagcggggccagaacgtgaccttcagatgcgaccccatcagcgagcacaaccggctgtactggtacaggcagaccctgggccagggccccgagttcctgacctactttcagaacgaggcccagctggaaaagtcccggctgctgagcgacagattcagcgccgaaagacccaagggcagcttcagcaccctggaaatccagcggaccgagcagggcgatagcgccatgtacctgtgtgccagcagcagcacaggcggccacaacgagcagttctttggccctggcacccggctgaccgtgctggaagatctgaagaacgtgttccccccagaggtggccgtgttcgagccttctgaggccgagatcagccacacccagaaagccaccctcgtgtgtctggccaccggcttctaccccgaccacgtggaactgtcttggtgggtcaacggcaaagaggtgcactccggcgtgtgcaccgatccccagcctctgaaagaacagcccgccctgaacgacagccggtactgcctgagcagcagactgagagtgtccgccaccttctggcagaacccccggaaccacttcagatgccaggtgcagttctacggcctgagcgagaacgacgagtggacccaggacagagccaagcccgtgacccagatcgtgtctgccgaagcctggggcagagccgattgcggctttaccagcgagagctaccagcagggcgtgctgagcgccaccatcctgtacgagatcctgctgggcaaggccaccctgtacgccgtgctggtgtctgccctggtgctgatggccatggtcaagcggaaggacagc

SEQ ID NO: 40 - DNA, 828 bp, Artificial Sequence
  Synthetic sequence TCR1,13 alpha chain (codon optimized; Cys modified)
atggaaacactgctgggcgtgtccctcgtgatcctgtggctgcagctggccagagtgaacagccagcagggggaagaggatccccaggccctgagcattcaggaaggcgagaacgccaccatgaactgcagctacaagaccagcatcaacaacctgcagtggtacagacagaacagcggcagaggcctggtgcacctgatcctgatcagaagcaacgagagagagaagcacagcggacggctgagagtgaccctggacacctccaagaagtccagctccctgctgatcaccgccagcagagccgccgataccgccagctacttctgtgccaccaagcgggattctggcgccggatcctaccagctgaccttcggcaagggcaccaagctgagcgtgatccccaacatccagaaccccgaccccgccgtgtatcagctgagagacagcaagagcagcgacaagagcgtgtgcctgttcaccgacttcgacagccagaccaacgtgtcccagagcaaggacagcgacgtgtacatcaccgataagtgcgtgctggacatgcggagcatggacttcaagagcaacagcgccgtggcctggtccaacaagagcgacttcgcctgcgccaacgccttcaacaacagcatcatccccgaggacacctttttccccagccccgagagcagctgcgacgtgaaactggtggagaagtccttcgagacagacaccaatctgaactttcagaacctgagcgtgatcggcttccggatcctgctgctgaaagtggccggcttcaatctgctgatgaccctgcggctgtggagcagctga

SEQ ID NO: 41 - DNA, 930 bp, Artificial Sequence
  Synthetic sequence TCR2,14 beta chain (codon optimized; Cys modified)
atgggcacctccctgctgtgttggatggccctgtgtctgctgggagccgaccatgccgatacaggggtgtcccaggacccccggcacaagattaccaagcggggccagaacgtgaccttcagatgcgaccccatcagcgagcacaaccggctgtactggtacaggcagaccctgggccagggccccgagttcctgacctactttcagaacgaggcccagctggaaaagtcccggctgctgagcgacagattcagcgccgaaagacccaagggcagcttcagcaccctggaaatccagcggaccgagcagggcgatagcgccatgtacctgtgtgccagcagcctcgtgaagggcgagaagctgttcttcggcagcggcacccagctgagcgtgctggaagatctgaacaaggtgttccccccagaggtggccgtgttcgagccttctgaggccgagatcagccacacccagaaagccaccctcgtgtgcctggccaccggctttttccccgaccacgtggaactgtcttggtgggtcaacggcaaagaggtgcactccggcgtgtgcaccgatccccagcctctgaaagaacagcccgccctgaacgacagccggtactgcctgagcagcagactgagagtgtccgccaccttctggcagaacccccggaaccacttcagatgccaggtgcagttctacggcctgagcgagaacgacgagtggacccaggacagagccaagcccgtgacccagatcgtgtctgccgaagcctggggcagagccgattgcggctttaccagcgtgtcctatcagcagggcgtgctgagcgccaccatcctgtacgagatcctgctgggcaaggccaccctgtacgccgtgctggtgtctgccctggtgctgatggccatggtcaagcggaaggactttggc

SEQ ID NO: 42 - DNA, 820 bp, Artificial Sequence
  Synthetic sequence TCR2,14 alpha chain (codon optimized; Cys modified)
atggaaacactgctgggcctgctgatcctgtggctgcagctgcagtgggtgtccagcaagcaggaagtgacacagatccctgccgccctgtctgtgcccgagggcgaaaatctggtgctgaactgcagcttcaccgacagcgccatctacaacctgcagtggttcagacaggaccccggcaagggcctgacaagcctgctgctgattcagagcagccagagagagcagaccagcggcagactgaacgccagcctggataagagcagcggccgcagcaccctgtatatcgccgcttctcagcctggcgactctgccacatatctgtgcgccgtgatcggcctgggcggcacctacaagtacatctttggcaccggcaccagactgaaagtgctggccaacatccagaaccccgaccccgccgtgtaccagctgagagacagcaagtccagcgacaagagcgtgtgtctgttcaccgacttcgacagccagaccaacgtgtcccagagcaaggacagcgacgtgtacatcaccgataagtgcgtgctggacatgcggagcatggacttcaagagcaacagcgccgtggcctggtccaacaagagcgacttcgcctgcgccaacgccttcaacaacagcatcatccccgaggacacctttttccccagccccgagagcagctgcgacgtgaaactggtggagaagtccttcgagacagacaccaatctgaactttcagaacctgagcgtgatcggcttccggatcctgctgctgaaagtggccggcttcaatctgctgatgaccctgcggctgtggagcagcg

SEQ ID NO: 43 - DNA, 933 bp, Artificial Sequence
  Synthetic sequence TCR5 beta chain (codon optimized; Cys modified)
atgggcacctccctgctgtgttggatggccctgtgtctgctgggagccgaccatgccgatacaggggtgtcccaggacccccggcacaagattaccaagcggggccagaacgtgaccttcagatgcgaccccatcagcgagcacaaccggctgtactggtacaggcagaccctgggccagggccccgagttcctgacctactttcagaacgaggcccagctggaaaagtcccggctgctgagcgacagattcagcgccgaaagacccaagggcagcttcagcaccctggaaatccagcggaccgagcagggggacagcgccatgtatctgtgtgccagctccctgaccaccctggacgagcagtatgtgggcccaggcaccagactgaccgtgaccgaggacctgaagaacgtgttccccccagaggtggccgtgttcgagccttctgaggccgagatcagccacacccagaaagccaccctcgtgtgtctggccaccggcttctaccccgatcacgtggagctgtcttggtgggtgaacggcaaagaggtgcacagcggcgtctgcaccgacccccagcccctgaaagagcagcccgccctgaacgacagccggtactgcctgagcagccggctgagagtgagcgccaccttctggcagaacccccggaaccacttccggtgccaggtgcagttctacggcctgagcgagaacgacgagtggacccaggacagagccaagcccgtgacccagatcgtgagcgccgaggcctggggcagagccgactgcggcttcaccagcgagagctaccagcagggcgtgctgtccgccacaatcctgtacgagatcctgctgggcaaggccaccctgtacgccgtgctggtgtccgccctggtgctgatggccatggtgaagcggaaggacagccggggc

SEQ ID NO: 44 - DNA, 816 bp, Artificial Sequence
  Synthetic sequence TCR5 alpha chain (codon optimized; Cys modified)
atggaaaccctgctgggcgtgtccctcgtgatcctgtggctgcagctggccagagtgaacagccagcagggcgaagaagatccccaggccctgagcatccaggaaggcgagaacgccacaatgaactgcagctacaagaccagcatcaacaacctgcagtggtacagacagaacagcggcagaggcctggtgcacctgatcctgatcagaagcaacgagagagagaagcactccggcagactgagagtgaccctggacaccagcaagaagtccagcagcctgctgatcaccgccagcagagccgccgataccgccagctacttctgcgccaccaactccggcaacacccccctggtgtttggcaagggcacccggctgagcgtgatcgccaacatccagaaccccgaccccgccgtgtaccagctgagagacagcaagagcagcgacaagagcgtgtgcctgttcaccgacttcgacagccagaccaacgtgtcccagagcaaggacagcgacgtgtacatcaccgataagtgcgtgctggacatgcggagcatggacttcaagagcaacagcgccgtggcctggtccaacaagagcgacttcgcctgcgccaacgccttcaacaacagcatcatccccgaggacacctttttccccagccccgagagcagctgcgacgtgaaactggtggagaagtccttcgagacagacaccaatctgaactttcagaacctgagcgtgatcggcttccggatcctgctgctgaaagtggccggcttcaatctgctgatgaccctgcggctgtggagcagctga

SEQ ID NO: 45 - DNA, 933 bp, Artificial Sequence
  Synthetic sequence TCR10 beta chain (codon optimized; Cys modified)
atgggcacctccctgctgtgttggatggccctgtgtctgctgggagccgaccatgccgatacaggggtgtcccaggacccccggcacaagattaccaagcggggccagaacgtgaccttcagatgcgaccccatcagcgagcacaaccggctgtactggtacaggcagaccctgggccagggccccgagttcctgacctactttcagaacgaggcccagctggaaaagtcccggctgctgagcgacagattcagcgccgaaagacccaagggcagcttcagcaccctggaaatccagcggaccgagcagggcgatagcgccatgtacctgtgcgccagctccatgctgaccaactacgagcagtacttcggccctggcacccggctgaccgtgaccgaggatctgaagaacgtgttccccccagaggtggccgtgttcgagccttctgaggccgagatcagccacacccagaaagccaccctcgtgtgtctggccaccggcttctaccccgaccacgtggaactgtcttggtgggtcaacggcaaagaggtgcactccggcgtgtgcaccgatccccagcctctgaaagaacagcccgccctgaacgacagccggtactgcctgagcagcagactgagagtgtccgccaccttctggcagaacccccggaaccacttcagatgccaggtgcagttctacggcctgagcgagaacgacgagtggacccaggacagagccaagcccgtgacccagatcgtgtctgccgaagcctggggcagagccgattgcggctttaccagcgagagctaccagcagggcgtgctgagcgccaccatcctgtacgagatcctgctgggcaaggccaccctgtacgccgtgctggtgtctgccctggtgctgatggccatggtcaagcggaaggacagcagaggc

SEQ ID NO: 46 - DNA, 828 bp, Artificial Sequence
  Synthetic sequence TCR10 alpha chain (codon optimized; Cys modified)
atgaagaagcacctgaccacctttctcgtgatcctgtggctgtacttctaccggggcaacggcaagaaccaggtggaacagagcccccagagcctgatcatcctggaaggcaagaattgcaccctgcagtgcaactacaccgtgtcccccttcagcaacctgcggtggtacaagcaggacaccggcagaggccctgtgtccctgaccatcatgaccttcagcgagaacaccaagagcaacggccggtacaccgccaccctggatgccgatacaaagcagagcagcctgcacatcaccgccagccagctgagcgattccgccagctacatctgcgtggtggattctggcggcggagccgatggcctgacatttggcaagggcacccacctgatcattcagccctacatccagaaccccgaccccgccgtgtaccagctgagagacagcaagtccagcgacaagagcgtgtgcctgttcaccgacttcgacagccagaccaacgtgtcccagagcaaggacagcgacgtgtacatcaccgataagtgcgtgctggacatgcggagcatggacttcaagagcaacagcgccgtggcctggtccaacaagagcgacttcgcctgcgccaacgccttcaacaacagcatcatccccgaggacacctttttccccagccccgagagcagctgcgacgtgaaactggtggagaagtccttcgagacagacaccaatctgaactttcagaacctgagcgtgatcggcttccggatcctgctgctgaaagtggccggcttcaatctgctgatgaccctgcggctgtggagcagctga

SEQ ID NO: 47 - DNA, 933 bp, Artificial Sequence
  Synthetic sequence TCR16 beta chain (codon optimized; Cys modified)
atgggcacctccctgctgtgttggatggccctgtgtctgctgggagccgaccatgccgatacaggggtgtcccaggacccccggcacaagattaccaagcggggccagaacgtgaccttcagatgcgaccccatcagcgagcacaaccggctgtactggtacaggcagaccctgggccagggccccgagttcctgacctactttcagaacgaggcccagctggaaaagtcccggctgctgagcgacagattcagcgccgaaagacccaagggcagcttcagcaccctggaaatccagcggaccgagcagggcgatagcgccatgtacctgtgtgccagcagcctggtcgtgggcaacgagcagtttttcggccctggcaccagactgaccgtgctggaagatctgaagaacgtgttccccccagaggtggccgtgttcgagccttctgaggccgagatcagccacacccagaaagccaccctcgtgtgtctggccaccggcttctaccccgaccacgtggaactgtcttggtgggtcaacggcaaagaggtgcactccggcgtgtgcaccgatccccagcctctgaaagaacagcccgccctgaacgacagccggtactgcctgagcagcagactgagagtgtccgccaccttctggcagaacccccggaaccacttcagatgccaggtgcagttctacggcctgagcgagaacgacgagtggacccaggacagagccaagcccgtgacccagatcgtgtctgccgaagcctggggcagagccgattgcggctttaccagcgagagctaccagcagggcgtgctgagcgccaccatcctgtacgagatcctgctgggcaaggccaccctgtacgccgtgctggtgtctgccctggtgctgatggccatggtcaagcggaaggacagcagaggc

SEQ ID NO: 48 - DNA, 819 bp, Artificial Sequence
  Synthetic sequence TCR16 alpha chain (codon optimized; Cys modified)
atggaaacactgctgggcctgctgatcctgtggctgcagctgcagtgggtgtccagcaagcaggaagtgacacagatccctgccgccctgtctgtgcccgagggcgaaaatctggtgctgaactgcagcttcaccgacagcgccatctacaacctgcagtggttcagacaggaccccggcaagggcctgacaagcctgctgctgattcagagcagccagagagagcagaccagcggcagactgaacgccagcctggataagagcagcggccgcagcaccctgtatatcgccgcttctcagcctggcgactctgccacatatctgtgcgccgtgcatctgctgaacgactacaagctgagcttcggagccggcaccaccgtgacagtgcgggccaacatccagaaccccgaccctgccgtgtaccagctgagagacagcaagtccagcgacaagagcgtgtgcctgttcaccgacttcgacagccagaccaacgtgtcccagagcaaggacagcgacgtgtacatcaccgataagtgcgtgctggacatgcggagcatggacttcaagagcaacagcgccgtggcctggtccaacaagagcgacttcgcctgcgccaacgccttcaacaacagcatcatccccgaggacacctttttccccagccccgagagcagctgcgacgtgaaactggtggagaagtccttcgagacagacaccaatctgaactttcagaacctgagcgtgatcggcttccggatcctgctgctgaaagtggccggcttcaatctgctgatgaccctgcggctgtggagcagctga

SEQ ID NO: 49 - DNA, 939 bp, Artificial Sequence
  Synthetic sequence TCR24 beta chain (wild type)
atgggtcctgggcttctccactggatggccctttgtctccttggaacaggtcatggggatgccatggtcatccagaacccaagataccaggttacccagtttggaaagccagtgaccctgagttgttctcagactttgaaccataacgtcatgtactggtaccagcagaagtcaagtcaggccccaaagctgctgttccactactatgacaaagattttaacaatgaagcagacacccctgataacttccaatccaggaggccgaacacttctttctgctttcttgacatccgctcaccaggcctgggggacgcagccatgtacctgtgtgccaccagcaagacacggatagctcaagagacccagtacttcgggccaggcacgcggctcctggtgctcgaggacctgaaaaacgtgttcccacccgaggtcgctgtgtttgagccatcagaagcagagatctcccacacccaaaaggccacactggtgtgcctggccacaggcttctaccccgaccacgtggagctgagctggtgggtgaatgggaaggaggtgcacagtggggtcagcacagacccgcagcccctcaaggagcagcccgccctcaatgactccagatactgcctgagcagccgcctgagggtctcggccaccttctggcagaacccccgcaaccacttccgctgtcaagtccagttctacgggctctcggagaatgacgagtggacccaggatagggccaaacctgtcacccagatcgtcagcgccgaggcctggggtagagcagactgtggcttcacctccgagtcttaccagcaaggggtcctgtctgccaccatcctctatgagatcttgctagggaaggccaccttgtatgccgtgctggtcagtgccctcgtgctgatggccatggtcaagagaaaggattccagaggctag

SEQ ID NO: 50 - DNA, 825 bp, Artificial Sequence
  Synthetic sequence TCR24 alpha chain (wild type)
atgctcctggagcttatcccactgctggggatacattttgtcctgagaactgccagagcccagtcagtgacccagcctgacatccacatcactgtctctgaaggagcctcactggagttgagatgtaactattcctatggggcaacaccttatctcttctggtatgtccagtcccccggccaaggcctccagctgctcctgaagtacttttcaggagacactctggttcaaggcattaaaggctttgaggctgaatttaagaggagtcaatcttccttcaacctgaggaaaccctctgtgcattggagtgatgctgctgagtacttctgtgctgtgggttataacaccaatgcaggcaaatcaacctttggggatgggactacgctcactgtgaagccaaatatccagaaccctgaccctgccgtgtaccagctgagagactctaaatccagtgacaagtctgtctgcctattcaccgattttgattctcaaacaaatgtgtcacaaagtaaggattctgatgtgtatatcacagacaaaactgtgctagacatgaggtctatggacttcaagagcaacagtgctgtggcctggagcaacaaatctgactttgcatgtgcaaacgccttcaacaacagcattattccagaagacaccttcttccccagcccagaaagttcctgtgatgtcaagctggtcgagaaaagctttgaaacagatacgaacctaaactttcaaaacctgtcagtgattgggttccgaatcctcctcctgaaagtggccgggtttaatctgctcatgacgctgcggctgtggtccagctga

SEQ ID NO: 51 - DNA, 929 bp, Artificial Sequence
  Synthetic sequence TCR29 beta chain (codon optimized; Cys modified)
atgggcacaagcctgctgtgttggatggccctgtgtctgctgggagccgatcatgccgatacgggagtgtcccaggatcctcggcacaagattaccaagcggggccagaacgtgaccttcagatgcgaccctatcagcgagcacaaccggctgtactggtacagacagacactcggccagggacctgagttcctgacctacttccagaacgaggcccagctggaaaagagcagactgctgagcgacagattcagcgccgaaagacccaagggcagcttcagcaccctggaaatccagagaaccgagcagggcgacagcgccatgtatctgtgtgccagctctctggtgtccggcaacaccatctacttcggcgaaggcagctggctgacagtggttaagatctgaacaaggtgttccccccagaggtggccgtgttcgagccttctgaggccgagatcagccacacccagaaagccaccctcgtgtgcctggccaccggctttttccccgaccacgtggaactgtcttggtgggtcaacggcaaagaggtgcactccggcgtgtgcaccgatccccagcctctgaaagaacagcccgccctgaacgacagccggtactgcctgagcagcagactgagagtgtccgccaccttctggcagaacccccggaaccacttcagatgccaggtgcagttctacggcctgagcgagaacgacgagtggacccaggacagagccaagcccgtgacccagatcgtgtctgccgaagcctggggcagagccgattgcggctttaccagcgtgtcctatcagcagggcgtgctgagcgccaccatcctgtacgagatcctgctgggcaaggccaccctgtacgccgtgctggtgtctgccctggtgctgatggccatggtcaagcggaaggactttggc

SEQ ID NO: 52 - DNA, 828 bp, Artificial Sequence
  Synthetic sequence TCR29 alpha chain (codon optimized; Cys modified)
atggaaacactgctgggcctgctgatcctgtggctgcaactgcaatgggtgtccagcaagcaagaagtgacacagatccctgccgctctgtctgtgcctgagggcgaaaacctggtgctgaactgcagcttcaccgacagcgccatctacaacctgcagtggttcagacaggaccccggcaagggactgacaagcctgctgctgattcagagcagccagagagagcagaccagcggcagactgaatgccagcctggataagtcctccggcagaagcaccctgtatatcgccgcttctcagcctggcgatagcgccacatatctgtgtgccgttagaggcggcaccacctccggcacctacaagtacatctttggcaccggcaccagactgaaggtgctggccaatatccagaaccccgaccccgccgtgtaccagctgagagacagcaagtccagcgacaagagcgtgtgtctgttcaccgacttcgacagccagaccaacgtgtcccagagcaaggacagcgacgtgtacatcaccgataagtgcgtgctggacatgcggagcatggacttcaagagcaacagcgccgtggcctggtccaacaagagcgacttcgcctgcgccaacgccttcaacaacagcatcatccccgaggacacctttttccccagccccgagagcagctgcgacgtgaaactggtggagaagtccttcgagacagacaccaatctgaactttcagaacctgagcgtgatcggcttccggatcctgctgctgaaagtggccggcttcaatctgctgatgaccctgcggctgtggagcagctga

SEQ ID NO: 53 - protein, 609 aa, Artificial Sequence
  Synthetic sequence TCR1,13 beta-P2A-alpha (Cys modified) with signal peptide
MGTSLLCWMALCLLGADHADTGVSQDPRHKITKRGQNVTFRCDPISEHNRLYWYRQTLGQGPEFLTYFQNEAQLEKSRLLSDRFSAERPKGSFSTLEIQRTEQGDSAMYLCASSSTGGHNEQFFGPGTRLTVLEDLKNVFPPEVAVFEPSEAEISHTQKATLVCLATGFYPDHVELSWWVNGKEVHSGVCTDPQPLKEQPALNDSRYCLSSRLRVSATFWQNPRNHFRCQVQFYGLSENDEWTQDRAKPVTQIVSAEAWGRADCGFTSESYQQGVLSATILYEILLGKATLYAVLVSALVLMAMVKRKDSRGGSGATNFSLLKQAGDVEENPGPMETLLGVSLVILWLQLARVNSQQGEEDPQALSIQEGENATMNCSYKTSINNLQWYRQNSGRGLVHLILIRSNEREKHSGRLRVTLDTSKKSSSLLITASRAADTASYFCATKRDSGAGSYQLTFGKGTKLSVIPNIQNPDPAVYQLRDSKSSDKSVCLFTDFDSQTNVSQSKDSDVYITDKCVLDMRSMDFKSNSAVAWSNKSDFACANAFNNSIIPEDTFFPSPESSCDVKLVEKSFETDTNLNFQNLSVIGFRILLLKVAGFNLLMTLRLWSS

SEQ ID NO: 54 - protein, 604 aa, Artificial Sequence
  Synthetic sequence TCR2,14 beta-P2A-alpha (Cys modified) with signal peptide
MGTSLLCWMALCLLGADHADTGVSQDPRHKITKRGQNVTFRCDPISEHNRLYWYRQTLGQGPEFLTYFQNEAQLEKSRLLSDRFSAERPKGSFSTLEIQRTEQGDSAMYLCASSLVKGEKLFFGSGTQLSVLEDLNKVFPPEVAVFEPSEAEISHTQKATLVCLATGFFPDHVELSWWVNGKEVHSGVCTDPQPLKEQPALNDSRYCLSSRLRVSATFWQNPRNHFRCQVQFYGLSENDEWTQDRAKPVTQIVSAEAWGRADCGFTSVSYQQGVLSATILYEILLGKATLYAVLVSALVLMAMVKRKDFGSGATNFSLLKQAGDVEENPGPMETLLGLLILWLQLQWVSSKQEVTQIPAALSVPEGENLVLNCSFTDSAIYNLQWFRQDPGKGLTSLLLIQSSQREQTSGRLNASLDKSSGRSTLYIAASQPGDSATYLCAVIGLGGTYKYIFGTGTRLKVLANIQNPDPAVYQLRDSKSSDKSVCLFTDFDSQTNVSQSKDSDVYITDKCVLDMRSMDFKSNSAVAWSNKSDFACANAFNNSIIPEDTFFPSPESSCDVKLVEKSFETDTNLNFQNLSVIGFRILLLKVAGFNLLMTLRLWSS

SEQ ID NO: 55 - protein, 604 aa, Artificial Sequence
  Synthetic sequence TCR5 beta-P2A-alpha (Cys modified) with signal peptide
MGTSLLCWMALCLLGADHADTGVSQDPRHKITKRGQNVTFRCDPISEHNRLYWYRQTLGQGPEFLTYFQNEAQLEKSRLLSDRFSAERPKGSFSTLEIQRTEQGDSAMYLCASSLTTLDEQYVGPGTRLTVTEDLKNVFPPEVAVFEPSEAEISHTQKATLVCLATGFYPDHVELSWWVNGKEVHSGVCTDPQPLKEQPALNDSRYCLSSRLRVSATFWQNPRNHFRCQVQFYGLSENDEWTQDRAKPVTQIVSAEAWGRADCGFTSESYQQGVLSATILYEILLGKATLYAVLVSALVLMAMVKRKDSRGGSGATNFSLLKQAGDVEENPGPMETLLGVSLVILWLQLARVNSQQGEEDPQALSIQEGENATMNCSYKTSINNLQWYRQNSGRGLVHLILIRSNEREKHSGRLRVTLDTSKKSSSLLITASRAADTASYFCATNSGNTPLVFGKGTRLSVIANIQNPDPAVYQLRDSKSSDKSVCLFTDFDSQTNVSQSKDSDVYITDKCVLDMRSMDFKSNSAVAWSNKSDFACANAFNNSIIPEDTFFPSPESSCDVKLVEKSFETDTNLNFQNLSVIGFRILLLKVAGFNLLMTLRLWSS

SEQ ID NO: 56 - protein, 608 aa, Artificial Sequence
  Synthetic sequence TCR10 beta-P2A-alpha (Cys modified) with signal peptide
MGTSLLCWMALCLLGADHADTGVSQDPRHKITKRGQNVTFRCDPISEHNRLYWYRQTLGQGPEFLTYFQNEAQLEKSRLLSDRFSAERPKGSFSTLEIQRTEQGDSAMYLCASSMLTNYEQYFGPGTRLTVTEDLKNVFPPEVAVFEPSEAEISHTQKATLVCLATGFYPDHVELSWWVNGKEVHSGVCTDPQPLKEQPALNDSRYCLSSRLRVSATFWQNPRNHFRCQVQFYGLSENDEWTQDRAKPVTQIVSAEAWGRADCGFTSESYQQGVLSATILYEILLGKATLYAVLVSALVLMAMVKRKDSRGGSGATNFSLLKQAGDVEENPGPMKKHLTTFLVILWLYFYRGNGKNQVEQSPQSLIILEGKNCTLQCNYTVSPFSNLRWYKQDTGRGPVSLTIMTFSENTKSNGRYTATLDADTKQSSLHITASQLSDSASYICVVDSGGGADGLTFGKGTHLIIQPYIQNPDPAVYQLRDSKSSDKSVCLFTDFDSQTNVSQSKDSDVYITDKCVLDMRSMDFKSNSAVAWSNKSDFACANAFNNSIIPEDTFFPSPESSCDVKLVEKSFETDTNLNFQNLSVIGFRILLLKVAGFNLLMTLRLWSS

SEQ ID NO: 57 - protein, 605 aa, Artificial Sequence
  Synthetic sequence TCR16 beta-P2A-alpha (Cys modified) with signal peptide
MGTSLLCWMALCLLGADHADTGVSQDPRHKITKRGQNVTFRCDPISEHNRLYWYRQTLGQGPEFLTYFQNEAQLEKSRLLSDRFSAERPKGSFSTLEIQRTEQGDSAMYLCASSLVVGNEQFFGPGTRLTVLEDLKNVFPPEVAVFEPSEAEISHTQKATLVCLATGFYPDHVELSWWVNGKEVHSGVCTDPQPLKEQPALNDSRYCLSSRLRVSATFWQNPRNHFRCQVQFYGLSENDEWTQDRAKPVTQIVSAEAWGRADCGFTSESYQQGVLSATILYEILLGKATLYAVLVSALVLMAMVKRKDSRGGSGATNFSLLKQAGDVEENPGPMETLLGLLILWLQLQWVSSKQEVTQIPAALSVPEGENLVLNCSFTDSAIYNLQWFRQDPGKGLTSLLLIQSSQREQTSGRLNASLDKSSGRSTLYIAASQPGDSATYLCAVHLLNDYKLSFGAGTTVTVRANIQNPDPAVYQLRDSKSSDKSVCLFTDFDSQTNVSQSKDSDVYITDKCVLDMRSMDFKSNSAVAWSNKSDFACANAFNNSIIPEDTFFPSPESSCDVKLVEKSFETDTNLNFQNLSVIGFRILLLKVAGFNLLMTLRLWSS

SEQ ID NO: 58 - protein, 585 aa, Artificial Sequence
  Synthetic sequence Consensus sequence of the TCR beta-P2A-alpha
MGTSLLCWMALCLLGADHADTGVSQDPRHKITKRGQNVTFRCDPISEHNRLYWYRQTLGQGPEFLTYFQNEAQLEKSRLLSDRFSAERPKGSFSTLEIQRTEQGDSAMYLCASSLVGEQFFGPGTRLTVLEDLKNVFPPEVAVFEPSEAEISHTQKATLVCLATGFYPDHVELSWWVNGKEVHSGVCTDPQPLKEQPALNDSRYCLSSRLRVSATFWQNPRNHFRCQVQFYGLSENDEWTQDRAKPVTQIVSAEAWGRADCGFTSESYQQGVLSATILYEILLGKATLYAVLVSALVLMAMVKRKDSRGGSGATNFSLLKQAGDVEENPGPMETLLGLVILWLQLRVNSKQQPQALSIEGENTLNCSYTSINLQWYRQDSGRGLVSLLLISSEREKTSGRLATLDSSKSSLITASQGDSASYLCAVSGGGYLTFGKGTRLSVLANIQNPDPAVYQLRDSKSSDKSVCLFTDFDSQTNVSQSKDSDVYITDKCVLDMRSMDFKSNSAVAWSNKSDFACANAFNNSIIPEDTFFPSPESSCDVKLVEKSFETDTNLNFQNLSVIGFRILLLKVAGFNLLMTLRLWSS

SEQ ID NO: 59 - DNA, 1830 bp, Artificial Sequence
  Synthetic sequence TCR1,13 beta-P2A-alpha (codon optimized; Cys modified)
atgggcacctccctgctgtgttggatggccctgtgtctgctgggagccgaccatgccgatacaggggtgtcccaggacccccggcacaagattaccaagcggggccagaacgtgaccttcagatgcgaccccatcagcgagcacaaccggctgtactggtacaggcagaccctgggccagggccccgagttcctgacctactttcagaacgaggcccagctggaaaagtcccggctgctgagcgacagattcagcgccgaaagacccaagggcagcttcagcaccctggaaatccagcggaccgagcagggcgatagcgccatgtacctgtgtgccagcagcagcacaggcggccacaacgagcagttctttggccctggcacccggctgaccgtgctggaagatctgaagaacgtgttccccccagaggtggccgtgttcgagccttctgaggccgagatcagccacacccagaaagccaccctcgtgtgtctggccaccggcttctaccccgaccacgtggaactgtcttggtgggtcaacggcaaagaggtgcactccggcgtgtgcaccgatccccagcctctgaaagaacagcccgccctgaacgacagccggtactgcctgagcagcagactgagagtgtccgccaccttctggcagaacccccggaaccacttcagatgccaggtgcagttctacggcctgagcgagaacgacgagtggacccaggacagagccaagcccgtgacccagatcgtgtctgccgaagcctggggcagagccgattgcggctttaccagcgagagctaccagcagggcgtgctgagcgccaccatcctgtacgagatcctgctgggcaaggccaccctgtacgccgtgctggtgtctgccctggtgctgatggccatggtcaagcggaaggacagcagaggcggaagcggcgccaccaacttcagcctgctgaaacaggccggcgacgtggaagagaaccctggccctatggaaacactgctgggcgtgtccctcgtgatcctgtggctgcagctggccagagtgaacagccagcagggggaagaggatccccaggccctgagcattcaggaaggcgagaacgccaccatgaactgcagctacaagaccagcatcaacaacctgcagtggtacagacagaacagcggcagaggcctggtgcacctgatcctgatcagaagcaacgagagagagaagcacagcggacggctgagagtgaccctggacacctccaagaagtccagctccctgctgatcaccgccagcagagccgccgataccgccagctacttctgtgccaccaagcgggattctggcgccggatcctaccagctgaccttcggcaagggcaccaagctgagcgtgatccccaacatccagaaccccgaccccgccgtgtatcagctgagagacagcaagagcagcgacaagagcgtgtgcctgttcaccgacttcgacagccagaccaacgtgtcccagagcaaggacagcgacgtgtacatcaccgataagtgcgtgctggacatgcggagcatggacttcaagagcaacagcgccgtggcctggtccaacaagagcgacttcgcctgcgccaacgccttcaacaacagcatcatccccgaggacacctttttccccagccccgagagcagctgcgacgtgaaactggtggagaagtccttcgagacagacaccaatctgaactttcagaacctgagcgtgatcggcttccggatcctgctgctgaaagtggccggcttcaatctgctgatgaccctgcggctgtggagcagctga

SEQ ID NO: 60 - DNA, 1813 bp, Artificial Sequence
  Synthetic sequence TCR2,14 beta-P2A-alpha (codon optimized; Cys modified)
atgggcacctccctgctgtgttggatggccctgtgtctgctgggagccgaccatgccgatacaggggtgtcccaggacccccggcacaagattaccaagcggggccagaacgtgaccttcagatgcgaccccatcagcgagcacaaccggctgtactggtacaggcagaccctgggccagggccccgagttcctgacctactttcagaacgaggcccagctggaaaagtcccggctgctgagcgacagattcagcgccgaaagacccaagggcagcttcagcaccctggaaatccagcggaccgagcagggcgatagcgccatgtacctgtgtgccagcagcctcgtgaagggcgagaagctgttcttcggcagcggcacccagctgagcgtgctggaagatctgaacaaggtgttccccccagaggtggccgtgttcgagccttctgaggccgagatcagccacacccagaaagccaccctcgtgtgcctggccaccggctttttccccgaccacgtggaactgtcttggtgggtcaacggcaaagaggtgcactccggcgtgtgcaccgatccccagcctctgaaagaacagcccgccctgaacgacagccggtactgcctgagcagcagactgagagtgtccgccaccttctggcagaacccccggaaccacttcagatgccaggtgcagttctacggcctgagcgagaacgacgagtggacccaggacagagccaagcccgtgacccagatcgtgtctgccgaagcctggggcagagccgattgcggctttaccagcgtgtcctatcagcagggcgtgctgagcgccaccatcctgtacgagatcctgctgggcaaggccaccctgtacgccgtgctggtgtctgccctggtgctgatggccatggtcaagcggaaggactttggcagcggcgccaccaacttcagcctgctgaaacaggccggcgacgtggaagagaaccctggccctaatctgaactttcagaacctgagcgtgatcggcttccggatcctgctgctgaaagtggccggcttcaatctgctgatgaccctgcggctgtggagcagcgatggaaacactgctgggcctgctgatcctgtggctgcagctgcagtgggtgtccagcaagcaggaagtgacacagatccctgccgccctgtctgtgcccgagggcgaaaatctggtgctgaactgcagcttcaccgacagcgccatctacaacctgcagtggttcagacaggaccccggcaagggcctgacaagcctgctgctgattcagagcagccagagagagcagaccagcggcagactgaacgccagcctggataagagcagcggccgcagcaccctgtatatcgccgcttctcagcctggcgactctgccacatatctgtgcgccgtgatcggcctgggcggcacctacaagtacatctttggcaccggcaccagactgaaagtgctggccaacatccagaaccccgaccccgccgtgtaccagctgagagacagcaagtccagcgacaagagcgtgtgtctgttcaccgacttcgacagccagaccaacgtgtcccagagcaaggacagcgacgtgtacatcaccgataagtgcgtgctggacatgcggagcatggacttcaagagcaacagcgccgtggcctggtccaacaagagcgacttcgcctgcgccaacgccttcaacaacagcatcatccccgaggacacctttttccccagccccgagagcagctgcgacgtgaaactggtggagaagtccttcgagacagacacc

SEQ ID NO: 61 - DNA, 1815 bp, Artificial Sequence
  Synthetic sequence TCR5 beta-P2A-alpha (codon optimized; Cys modified)
atgggcacctccctgctgtgttggatggccctgtgtctgctgggagccgaccatgccgatacaggggtgtcccaggacccccggcacaagattaccaagcggggccagaacgtgaccttcagatgcgaccccatcagcgagcacaaccggctgtactggtacaggcagaccctgggccagggccccgagttcctgacctactttcagaacgaggcccagctggaaaagtcccggctgctgagcgacagattcagcgccgaaagacccaagggcagcttcagcaccctggaaatccagcggaccgagcagggggacagcgccatgtatctgtgtgccagctccctgaccaccctggacgagcagtatgtgggcccaggcaccagactgaccgtgaccgaggacctgaagaacgtgttccccccagaggtggccgtgttcgagccttctgaggccgagatcagccacacccagaaagccaccctcgtgtgtctggccaccggcttctaccccgatcacgtggagctgtcttggtgggtgaacggcaaagaggtgcacagcggcgtctgcaccgacccccagcccctgaaagagcagcccgccctgaacgacagccggtactgcctgagcagccggctgagagtgagcgccaccttctggcagaacccccggaaccacttccggtgccaggtgcagttctacggcctgagcgagaacgacgagtggacccaggacagagccaagcccgtgacccagatcgtgagcgccgaggcctggggcagagccgactgcggcttcaccagcgagagctaccagcagggcgtgctgtccgccacaatcctgtacgagatcctgctgggcaaggccaccctgtacgccgtgctggtgtccgccctggtgctgatggccatggtgaagcggaaggacagccggggcggcagcggcgccaccaacttcagcctgctgaagcaggccggcgacgtggaggaaaaccctggccccatggaaaccctgctgggcgtgtccctcgtgatcctgtggctgcagctggccagagtgaacagccagcagggcgaagaagatccccaggccctgagcatccaggaaggcgagaacgccacaatgaactgcagctacaagaccagcatcaacaacctgcagtggtacagacagaacagcggcagaggcctggtgcacctgatcctgatcagaagcaacgagagagagaagcactccggcagactgagagtgaccctggacaccagcaagaagtccagcagcctgctgatcaccgccagcagagccgccgataccgccagctacttctgcgccaccaactccggcaacacccccctggtgtttggcaagggcacccggctgagcgtgatcgccaacatccagaaccccgaccccgccgtgtaccagctgagagacagcaagagcagcgacaagagcgtgtgcctgttcaccgacttcgacagccagaccaacgtgtcccagagcaaggacagcgacgtgtacatcaccgataagtgcgtgctggacatgcggagcatggacttcaagagcaacagcgccgtggcctggtccaacaagagcgacttcgcctgcgccaacgccttcaacaacagcatcatccccgaggacacctttttccccagccccgagagcagctgcgacgtgaaactggtggagaagtccttcgagacagacaccaatctgaactttcagaacctgagcgtgatcggcttccggatcctgctgctgaaagtggccggcttcaatctgctgatgaccctgcggctgtggagcagctga

SEQ ID NO: 62 - DNA, 1827 bp, Artificial Sequence
  Synthetic sequence TCR10 beta P2A-alpha (codon optimized; Cys modified)
atgggcacctccctgctgtgttggatggccctgtgtctgctgggagccgaccatgccgatacaggggtgtcccaggacccccggcacaagattaccaagcggggccagaacgtgaccttcagatgcgaccccatcagcgagcacaaccggctgtactggtacaggcagaccctgggccagggccccgagttcctgacctactttcagaacgaggcccagctggaaaagtcccggctgctgagcgacagattcagcgccgaaagacccaagggcagcttcagcaccctggaaatccagcggaccgagcagggcgatagcgccatgtacctgtgcgccagctccatgctgaccaactacgagcagtacttcggccctggcacccggctgaccgtgaccgaggatctgaagaacgtgttccccccagaggtggccgtgttcgagccttctgaggccgagatcagccacacccagaaagccaccctcgtgtgtctggccaccggcttctaccccgaccacgtggaactgtcttggtgggtcaacggcaaagaggtgcactccggcgtgtgcaccgatccccagcctctgaaagaacagcccgccctgaacgacagccggtactgcctgagcagcagactgagagtgtccgccaccttctggcagaacccccggaaccacttcagatgccaggtgcagttctacggcctgagcgagaacgacgagtggacccaggacagagccaagcccgtgacccagatcgtgtctgccgaagcctggggcagagccgattgcggctttaccagcgagagctaccagcagggcgtgctgagcgccaccatcctgtacgagatcctgctgggcaaggccaccctgtacgccgtgctggtgtctgccctggtgctgatggccatggtcaagcggaaggacagcagaggcggaagcggcgccaccaacttcagcctgctgaaacaggccggcgacgtggaagagaaccctggccccatgaagaagcacctgaccacctttctcgtgatcctgtggctgtacttctaccggggcaacggcaagaaccaggtggaacagagcccccagagcctgatcatcctggaaggcaagaattgcaccctgcagtgcaactacaccgtgtcccccttcagcaacctgcggtggtacaagcaggacaccggcagaggccctgtgtccctgaccatcatgaccttcagcgagaacaccaagagcaacggccggtacaccgccaccctggatgccgatacaaagcagagcagcctgcacatcaccgccagccagctgagcgattccgccagctacatctgcgtggtggattctggcggcggagccgatggcctgacatttggcaagggcacccacctgatcattcagccctacatccagaaccccgaccccgccgtgtaccagctgagagacagcaagtccagcgacaagagcgtgtgcctgttcaccgacttcgacagccagaccaacgtgtcccagagcaaggacagcgacgtgtacatcaccgataagtgcgtgctggacatgcggagcatggacttcaagagcaacagcgccgtggcctggtccaacaagagcgacttcgcctgcgccaacgccttcaacaacagcatcatccccgaggacacctttttccccagccccgagagcagctgcgacgtgaaactggtggagaagtccttcgagacagacaccaatctgaactttcagaacctgagcgtgatcggcttccggatcctgctgctgaaagtggccggcttcaatctgctgatgaccctgcggctgtggagcagctga

SEQ ID NO: 63 - DNA, 1818 bp, Artificial Sequence
  Synthetic sequence TCR16 beta-P2A-alpha (codon optimized; Cys modified)
atgggcacctccctgctgtgttggatggccctgtgtctgctgggagccgaccatgccgatacaggggtgtcccaggacccccggcacaagattaccaagcggggccagaacgtgaccttcagatgcgaccccatcagcgagcacaaccggctgtactggtacaggcagaccctgggccagggccccgagttcctgacctactttcagaacgaggcccagctggaaaagtcccggctgctgagcgacagattcagcgccgaaagacccaagggcagcttcagcaccctggaaatccagcggaccgagcagggcgatagcgccatgtacctgtgtgccagcagcctggtcgtgggcaacgagcagtttttcggccctggcaccagactgaccgtgctggaagatctgaagaacgtgttccccccagaggtggccgtgttcgagccttctgaggccgagatcagccacacccagaaagccaccctcgtgtgtctggccaccggcttctaccccgaccacgtggaactgtcttggtgggtcaacggcaaagaggtgcactccggcgtgtgcaccgatccccagcctctgaaagaacagcccgccctgaacgacagccggtactgcctgagcagcagactgagagtgtccgccaccttctggcagaacccccggaaccacttcagatgccaggtgcagttctacggcctgagcgagaacgacgagtggacccaggacagagccaagcccgtgacccagatcgtgtctgccgaagcctggggcagagccgattgcggctttaccagcgagagctaccagcagggcgtgctgagcgccaccatcctgtacgagatcctgctgggcaaggccaccctgtacgccgtgctggtgtctgccctggtgctgatggccatggtcaagcggaaggacagcagaggcggaagcggcgccaccaacttcagcctgctgaaacaggccggcgacgtggaagagaaccctggccctatggaaacactgctgggcctgctgatcctgtggctgcagctgcagtgggtgtccagcaagcaggaagtgacacagatccctgccgccctgtctgtgcccgagggcgaaaatctggtgctgaactgcagcttcaccgacagcgccatctacaacctgcagtggttcagacaggaccccggcaagggcctgacaagcctgctgctgattcagagcagccagagagagcagaccagcggcagactgaacgccagcctggataagagcagcggccgcagcaccctgtatatcgccgcttctcagcctggcgactctgccacatatctgtgcgccgtgcatctgctgaacgactacaagctgagcttcggagccggcaccaccgtgacagtgcgggccaacatccagaaccccgaccctgccgtgtaccagctgagagacagcaagtccagcgacaagagcgtgtgcctgttcaccgacttcgacagccagaccaacgtgtcccagagcaaggacagcgacgtgtacatcaccgataagtgcgtgctggacatgcggagcatggacttcaagagcaacagcgccgtggcctggtccaacaagagcgacttcgcctgcgccaacgccttcaacaacagcatcatccccgaggacacctttttccccagccccgagagcagctgcgacgtgaaactggtggagaagtccttcgagacagacaccaatctgaactttcagaacctgagcgtgatcggcttccggatcctgctgctgaaagtggccggcttcaatctgctgatgaccctgcggctgtggagcagctga

SEQ ID NO: 64 - protein, 1135 aa, Artificial Sequence
  Synthetic sequence HMHA1 (wt)
MFSRKKRELMKTPSISKKNRAGSPSPQPSGELPRKDGADAVFPGPSLEPPAGSSGVKATGTLKRPTSLSRHASAAGFPLSGAASWTLGRSHRSPLTAASPGELPTEGAGPDVVEDISHLLADVARFAEGLEKLKECVLRDDLLEARRPRAHECLGEALRVMHQIISKYPLLNTVETLTAAGTLIAKVKAFHYESNNDLEKQEFEKALETIAVAFSSTVSEFLMGEVDSSTLLAVPPGDSSQSMESLYGPGSEGTPPSLEDCDAGCLPAEEVDVLLQRCEGGVDAALLYAKNMAKYMKDLISYLEKRTTLEMEFAKGLQKIAHNCRQSVMQEPHMPLLSIYSLALEQDLEFGHSMVQAVGTLQTQTFMQPLTLRRLEHEKRRKEIKEAWHRQRKLQEAESNLRKAKQGYVQRCEDHDKARFLVAKAEEEQAGSAPGAGSTATKTLDKRRRLEEEAKNKAEEAMATYRTCVADAKTQKQELEDTKVTALRQIQEVIRQSDQTIKSATISYYQMMHMQTAPLPVHFQMLCESSKLYDPGQQYASHVRQLQRDQEPDVHYDFEPHVSANAWSPVMRARKSSFNVSDVARPEAAGSPPEEGGCTEGTPAKDHRAGRGHQVHKSWPLSISDSDSGLDPGPGAGDFKKFERTSSSGTMSSTEELVDPDGGAGASAFEQADLNGMTPELPVAVPSGPFRHEGLSKAARTHRLRKLRTPAKCRECNSYVYFQGAECEECCLACHKKCLETLAIQCGHKKLQGRLQLFGQDFSHAARSAPDGVPFIVKKCVCEIERRALRTKGIYRVNGVKTRVEKLCQAFENGKELVELSQASPHDISNVLKLYLRQLPEPLISFRLYHELVGLAKDSLKAEAEAKAASRGRQDGSESEAVAVALAGRLRELLRDLPPENRASLQYLLRHLRRIVEVEQDNKMTPGNLGIVFGPTLLRPRPTEATVSLSSLVDYPHQARVIETLIVHYGLVFEEEPEETPGGQDESSNQRAEVVVQVPYLEAGEAVVYPLQEAAADGCRESRVVSNDSDSDLEEASELLSSSEASALGHLSFLEQQQSEASLEVASGSHSGSEEQLEATAREDGDGDEDGPAQQLSGFNTNQSNNVLQAPLPPMRLRGGRMTLGSCRERQPEFV

SEQ ID NO: 65 - protein, 9 aa, Artificial Sequence
  Synthetic sequence HA-1 non-immunogenic peptide wild type
VLRDDLLEA

SEQ ID NO: 66 - protein, 9 aa, Artificial Sequence
  Synthetic sequence HA-1H antigen polymorphism
VLHDDLLEA

SEQ ID NO: 67 - DNA, 1206 bp, Artificial Sequence
  Synthetic sequence Inducible Caspase9 (codon optimized)
atgctggaaggcgtgcaggtggaaaccatcagccctggcgacggcagaaccttccctaagaggggccagacctgcgtggtgcactacaccggaatgctggaagatggcaagaaggtggacagcagccgggaccggaacaagcccttcaagttcatgctgggcaagcaggaagtgatccggggctgggaagagggcgtggcccagatgtctgtgggccagagagccaagctgaccatctcccccgattacgcctacggcgccacaggccaccctggcatcattcctccacacgccacactggtgttcgacgtggaactgctgaagctggaaagcggcggaggcagcggagtggatggctttggagatgtgggcgccctggaaagcctgagaggcaatgccgacctggcctacatcctgagcatggaaccttgcggccactgcctgattatcaacaacgtgaacttctgcagagagagcggcctgcggaccagaaccggcagcaacatcgactgcgagaagctgcggcggagattcagcagcctgcacttcatggtggaagtgaagggcgacctgaccgccaagaaaatggtgctggccctgctggaactggcccagcaggatcatggcgctctggactgctgtgtggtcgtgatcctgagccacggctgccaggccagccatctgcagttccctggcgccgtgtatggcaccgatggctgtcctgtgtccgtggaaaagatcgtgaacatcttcaacggcaccagctgccccagcctgggcggaaagcccaagctgttctttattcaagcctgcggaggcgagcagaaggaccacggatttgaggtggcctccaccagccccgaggatgagagccctggaagcaaccctgagcccgacgccaccccatttcaggaaggcctgagaaccttcgaccagctggacgccatcagctccctgcccacccccagcgatatcttcgtgtcctacagcaccttccccggctttgtgtcctggcgggatcccaagtccggctcttggtacgtggaaaccctggacgacatcttcgagcagtgggcccatagcgaggacctgcagagcctgctgctgagagtggccaatgccgtgtccgtgaagggcatctacaagcagatgcctggctgcttcaacttcctgcggaagaagctgtttttcaagaccagcgccagc

SEQ ID NO: 68 - DNA, 159 bp, Artificial Sequence
  Synthetic sequence RQR (codon optimized)
gcctgcccctacagcaaccctagcctgtgttctggcggcggaggcagcgaactgcctacccagggcaccttcagcaacgtgtccaccaatgtgtctggcggaggcggctctgcctgcccttactccaatccatccctgtgcagcggagggggcggaagc

SEQ ID NO: 69 - protein, 53 aa, Artificial Sequence
  Synthetic sequence RQR
ACPYSNPSLCSGGGGSELPTQGTFSNVSTNVSGGGGSACPYSNPSLCSGGGGS

SEQ ID NO: 70 - protein, 235 aa, Artificial Sequence
  Synthetic sequence CD8 co-receptor alpha chain with signal peptide
MALPVTALLLPLALLLHAARPSQFRVSPLDRTWNLGETVELKCQVLLSNPTSGCSWLFQPRGAAASPTFLLYLSQNKPKAAEGLDTQRFSGKRLGDTFVLTLSDFRRENEGYYFCSALSNSIMYFSHFVPVFLPAKPTTTPAPRPPTPAPTIASQPLSLRPEACRPAAGGAVHTRGLDFACDIYIWAPLAGTCGVLLLSLVITLYCNHRNRRRVCKCPRPVVKSGDKPSLSARYV

SEQ ID NO: 71 - protein, 210 aa, Artificial Sequence
  Synthetic sequence CD8 co-receptor beta chain isoform 1 with signal peptide
MRPRLWLLLAAQLTVLHGNSVLQQTPAYIKVQTNKMVMLSCEAKISLSNMRIYWLRQRQAPSSDSHHEFLALWDSAKGTIHGEEVEQEKIAVFRDASRFILNLTSVKPEDSGIYFCMIVGSPELTFGKGTQLSVVDFLPTTAQPTKKSTLKKRVCRLPRPETQKGPLCSPITLGLLVAGVLVLLVSLGVAIHLCCRRRRARLRFMKQFYK

SEQ ID NO: 72 - protein, 221 aa, Artificial Sequence
  Synthetic sequence CD8 co-receptor beta chain isoform 2 with signal peptide
MRPRLWLLLAAQLTVLHGNSVLQQTPAYIKVQTNKMVMLSCEAKISLSNMRIYWLRQRQAPSSDSHHEFLALWDSAKGTIHGEEVEQEKIAVFRDASRFILNLTSVKPEDSGIYFCMIVGSPELTFGKGTQLSVVDFLPTTAQPTKKSTLKKRVCRLPRPETQKGPLCSPITLGLLVAGVLVLLVSLGVAIHLCCRRRRARLRFMKQLRLHPLEKCSRMDY

SEQ ID NO: 73 - protein, 246 aa, Artificial Sequence
  Synthetic sequence CD8 co-receptor beta chain isoform 3 with signal peptide
MRPRLWLLLAAQLTVLHGNSVLQQTPAYIKVQTNKMVMLSCEAKISLSNMRIYWLRQRQAPSSDSHHEFLALWDSAKGTIHGEEVEQEKIAVFRDASRFILNLTSVKPEDSGIYFCMIVGSPELTFGKGTQLSVVDFLPTTAQPTKKSTLKKRVCRLPRPETQKGPLCSPITLGLLVAGVLVLLVSLGVAIHLCCRRRRARLRFMKQKFNIVCLKISGFTTCCCFQILQISREYGFGVLLQKDIGQ

SEQ ID NO: 74 - protein, 246 aa, Artificial Sequence; identical to SEQ ID NO: 73
  Synthetic sequence CD8 co-receptor beta chain isoform 4 with signal peptide

SEQ ID NO: 75 - protein, 243 aa, Artificial Sequence
  Synthetic sequence CD8 co-receptor beta chain isoform 5 with signal peptide
MRPRLWLLLAAQLTVLHGNSVLQQTPAYIKVQTNKMVMLSCEAKISLSNMRIYWLRQRQAPSSDSHHEFLALWDSAKGTIHGEEVEQEKIAVFRDASRFILNLTSVKPEDSGIYFCMIVGSPELTFGKGTQLSVVDFLPTTAQPTKKSTLKKRVCRLPRPETQKGPLCSPITLGLLVAGVLVLLVSLGVAIHLCCRRRRARLRFMKQPQGEGISGTFVPQCLHGYYSNTTTSQKLLNPWILKT

SEQ ID NO: 76 - DNA, 66 bp, Artificial Sequence
  Synthetic sequence P2A-1 (codon-optimized)
ggaagtggagctacgaatttttctttattaaaacaagcaggagatgttgaggagaatcccggtcca

SEQ ID NO: 77 - DNA, 63 bp, Artificial Sequence
  Synthetic sequence P2A-2 (codon-optimized)
agcggcgccaccaacttcagcctgctgaaacaggccggcgacgtggaagagaaccctggccct

SEQ ID NO: 78 - DNA, 65 bp, Artificial Sequence
  Synthetic sequence P2A-3 (codon-optimized)
gaagcggcgccacaaatttcagcctgctgaagcaggccggcgacgtggaagagaaccctggccct

SEQ ID NO: 79 - DNA, 66 bp, Artificial Sequence
  Synthetic sequence P2A-4 (codon-optimized)
ggctccggcgccaccaacttttcactgctgaaacaggctggggatgtggaagaaaatcccggccca

SEQ ID NO: 80 - DNA, 66 bp, Artificial Sequence
  Synthetic sequence P2A-5
ggcagcggcgccaccaactttagcctgctgaaacaggctggcgacgtggaagagaaccccggacct

SEQ ID NO: 81 - DNA, 66 bp, Artificial Sequence
  Synthetic sequence P2A-6
ggctctggcgccaccaactttagcctgctgaaacaggctggcgacgtggaagagaaccccggacct

SEQ ID NO: 82 - DNA, 63 bp, Artificial Sequence
  Synthetic sequence T2A
ggaagcggagagggcagaggaagtctgctaacatgcggtgacgtcgaggagaatcctggacct

SEQ ID NO: 83 - DNA, 69 bp, Artificial Sequence
  Synthetic sequence E2A
ggaagcggacagtgtactaattatgctctcttgaaattggctggagatgttgagagcaaccctggacct

SEQ ID NO: 84 - DNA, 75 bp, Artificial Sequence
  Synthetic sequence F2A
ggaagcggagtgaaacagactttgaattttgaccttctcaagttggcgggagacgtggagtccaaccctggacct

SEQ ID NO: 85 - DNA, 4713 bp, Artificial Sequence
  Synthetic sequence iC9-HA1-TCR2-RQR-CD8
atgctggaaggcgtgcaggtggaaaccatcagccctggcgacggcagaaccttccctaagaggggccagacctgcgtggtgcactacaccggaatgctggaagatggcaagaaggtggacagcagccgggaccggaacaagcccttcaagttcatgctgggcaagcaggaagtgatccggggctgggaagagggcgtggcccagatgtctgtgggccagagagccaagctgaccatctcccccgattacgcctacggcgccacaggccaccctggcatcattcctccacacgccacactggtgttcgacgtggaactgctgaagctggaaagcggcggaggcagcggagtggatggctttggagatgtgggcgccctggaaagcctgagaggcaatgccgacctggcctacatcctgagcatggaaccttgcggccactgcctgattatcaacaacgtgaacttctgcagagagagcggcctgcggaccagaaccggcagcaacatcgactgcgagaagctgcggcggagattcagcagcctgcacttcatggtggaagtgaagggcgacctgaccgccaagaaaatggtgctggccctgctggaactggcccagcaggatcatggcgctctggactgctgtgtggtcgtgatcctgagccacggctgccaggccagccatctgcagttccctggcgccgtgtatggcaccgatggctgtcctgtgtccgtggaaaagatcgtgaacatcttcaacggcaccagctgccccagcctgggcggaaagcccaagctgttctttattcaagcctgcggaggcgagcagaaggaccacggatttgaggtggcctccaccagccccgaggatgagagccctggaagcaaccctgagcccgacgccaccccatttcaggaaggcctgagaaccttcgaccagctggacgccatcagctccctgcccacccccagcgatatcttcgtgtcctacagcaccttccccggctttgtgtcctggcgggatcccaagtccggctcttggtacgtggaaaccctggacgacatcttcgagcagtgggcccatagcgaggacctgcagagcctgctgctgagagtggccaatgccgtgtccgtgaagggcatctacaagcagatgcctggctgcttcaacttcctgcggaagaagctgtttttcaagaccagcgccagcggaagtggagctacgaatttttctttattaaaacaagcaggagatgttgaggagaatcccggtccaatgggcacctccctgctgtgttggatggccctgtgtctgctgggagccgaccatgccgatacaggggtgtcccaggacccccggcacaagattaccaagcggggccagaacgtgaccttcagatgcgaccccatcagcgagcacaaccggctgtactggtacaggcagaccctgggccagggccccgagttcctgacctactttcagaacgaggcccagctggaaaagtcccggctgctgagcgacagattcagcgccgaaagacccaagggcagcttcagcaccctggaaatccagcggaccgagcagggcgatagcgccatgtacctgtgtgccagcagcctcgtgaagggcgagaagctgttcttcggcagcggcacccagctgagcgtgctggaagatctgaacaaggtgttccccccagaggtggccgtgttcgagccttctgaggccgagatcagccacacccagaaagccaccctcgtgtgcctggccaccggctttttccccgaccacgtggaactgtcttggtgggtcaacggcaaagaggtgcactccggcgtgtgcaccgatccccagcctctgaaagaacagcccgccctgaacgacagccggtactgcctgagcagcagactgagagtgtccgccaccttctggcagaacccccggaaccacttcagatgccaggtgcagttctacggcctgagcgagaacgacgagtggacccaggacagagccaagcccgtgacccagatcgtgtctgccgaagcctggggcagagccgattgcggctttaccagcgtgtcctatcagcagggcgtgctgagcgccaccatcctgtacgagatcctgctgggcaaggccaccctgtacgccgtgctggtgtctgccctggtgctgatggccatggtcaagcggaaggactttggcagcggcgccaccaacttcagcctgctgaaacaggccggcgacgtggaagagaaccctggccctatggaaacactgctgggcctgctgatcctgtggctgcagctgcagtgggtgtccagcaagcaggaagtgacacagatccctgccgccctgtctgtgcccgagggcgaaaatctggtgctgaactgcagcttcaccgacagcgccatctacaacctgcagtggttcagacaggaccccggcaagggcctgacaagcctgctgctgattcagagcagccagagagagcagaccagcggcagactgaacgccagcctggataagagcagcggccgcagcaccctgtatatcgccgcttctcagcctggcgactctgccacatatctgtgcgccgtgatcggcctgggcggcacctacaagtacatctttggcaccggcaccagactgaaagtgctggccaacatccagaaccccgaccccgccgtgtaccagctgagagacagcaagtccagcgacaagagcgtgtgtctgttcaccgacttcgacagccagaccaacgtgtcccagagcaaggacagcgacgtgtacatcaccgataagtgcgtgctggacatgcggagcatggacttcaagagcaacagcgccgtggcctggtccaacaagagcgacttcgcctgcgccaacgccttcaacaacagcatcatccccgaggacacctttttccccagccccgagagcagctgcgacgtgaaactggtggagaagtccttcgagacagacaccaatctgaactttcagaacctgagcgtgatcggcttccggatcctgctgctgaaagtggccggcttcaatctgctgatgaccctgcggctgtggagcagcggaagcggcgccacaaatttcagcctgctgaagcaggccggcgacgtggaagagaaccctggccctatgaggcccagactgtggctgctgctggccgctcagctgacagtgctgcacggcaatagcgtggcctgcccctacagcaaccctagcctgtgttctggcggcggaggcagcgaactgcctacccagggcaccttcagcaacgtgtccaccaatgtgtctggcggaggcggctctgcctgcccttactccaatccatccctgtgcagcggagggggcggaagcctgcagcagacaccagcctacatcaaggtgcagaccaacaagatggtcatgctgagctgcgaggccaagatcagcctgagcaacatgcggatctactggctgcggcagagacaggcccctagcagcgatagccaccacgagtttctggccctgtgggacagcgccaagggcaccattcacggcgaggaagtggaacaggaaaagatcgccgtgttccgggacgccagccggttcatcctgaacctgaccagcgtgaagcccgaggactccggcatctatttctgcatgatcgtgggctcccccgagctgaccttcggcaagggaacacagctgtccgtggtggacttcctgcctaccacagcccagcccaccaagaagtctaccctgaagaaaagagtgtgccggctgcccagacccgagacacagaaaggccctctgtgcagccctatcaccctgggactgctggtggctggcgtgctggtgctgctggtgtctctgggagtggccatccacctgtgctgcagaagaaggcgggccagactgcggttcatgaagcagttctacaagggctccggcgccaccaacttttcactgctgaaacaggctggggatgtggaagaaaatcccggcccaatggccctgcctgtgaccgctctgctgctgcctctggcactgctgctgcatgccgccagacccagccagttcagagtgtcccccctggacagaacctggaacctgggcgagacagtggaactgaagtgccaggtgctgctgagcaaccccaccagcggctgcagctggctgttccagcctagaggcgctgccgccagccctacctttctgctgtacctgagccagaacaagcccaaggccgccgagggcctggacacccagagattcagcggcaagagactgggcgacaccttcgtgctgaccctgtccgacttcagaagagagaacgagggctactacttctgctccgccctgagcaatagcatcatgtacttcagccacttcgtgcccgtgtttctgcccgccaagcctacaaccacccctgccccaagacctcccacacccgcccctacaattgccagccagcctctgtctctgaggcccgaggcttgtagaccagctgctggcggagccgtgcacaccagaggactggactttgcctgcgacatctacatctgggcccctctggccggcacttgcggagtgctgctgctgagtctcgtgatcaccctgtactgcaaccaccggaaccggcggagagtgtgcaagtgccctaggcccgtcgtgaagtccggcgacaagccttctctgagcgccagatatgtctga

SEQ ID NO: 86 - protein, 13 aa, Artificial Sequence
  Synthetic sequence TCR29 beta chain CDR3
CASSLVSGNTIYF

SEQ ID NO: 87 - protein, 15 aa, Artificial Sequence
  Synthetic sequence TCR1 alpha chain CDR3
CATKRDSGAGSYQLT

SEQ ID NO: 88 - protein, 14 aa, Artificial Sequence
  Synthetic sequence TCR2 alpha chain CDR3
CAVIGLGGTYKYIF

SEQ ID NO: 89 - protein, 12 aa, Artificial Sequence
  Synthetic sequence TCR5 alpha chain CDR3
CATNSGNTPLVF

SEQ ID NO: 90 - protein, 14 aa, Artificial Sequence
  Synthetic sequence TCR10 alpha chain CDR3
CVVDSGGGADGLTF

SEQ ID NO: 91 - protein, 13 aa, Artificial Sequence
  Synthetic sequence TCR16 alpha chain CDR3
CAVHLLNDYKLSF

SEQ ID NO: 92 - protein, 16 aa, Artificial Sequence
  Synthetic sequence TCR29 alpha chain CDR3
CAVRGGTTSGTYKYIF

SEQ ID NO: 93 - DNA, 21 bp, Artificial Sequence
  TCR alpha-chain primer
ggtgaataggcagacagactt

SEQ ID NO: 94 - DNA, 20 bp, Artificial Sequence
  TCR beta-chain primer
gtggccaggcacaccagtgt

SEQ ID NO: 95 - protein, 402 aa, Artificial Sequence
  Synthetic sequence inducible caspase-9
MLEGVQVETISPGDGRTFPKRGQTCVVHYTGMLEDGKKVDSSRDRNKPFKFMLGKQEVIRGWEEGVAQMSVGQRAKLTISPDYAYGATGHPGIIPPHATLVFDVELLKLESGGGSGVDGFGDVGALESLRGNADLAYILSMEPCGHCLIINNVNFCRESGLRTRTGSNIDCEKLRRRFSSLHFMVEVKGDLTAKKMVLALLELAQQDHGALDCCVVVILSHGCQASHLQFPGAVYGTDGCPVSVEKIVNIFNGTSCPSLGGKPKLFFIQACGGEQKDHGFEVASTSPEDESPGSNPEPDATPFQEGLRTFDQLDAISSLPTPSDIFVSYSTFPGFVSWRDPKSGSWYVETLDDIFEQWAHSEDLQSLLLRVANAVSVKGIYKQMPGCFNFLRKKLFFKTSAS

SEQ ID NO: 96 - protein, 112 aa, Artificial Sequence
  Synthetic sequence TCR1,13 beta chain variable region (mature)
GVSQDPRHKITKRGQNVTFRCDPISEHNRLYWYRQTLGQGPEFLTYFQNEAQLEKSRLLSDRFSAERPKGSFSTLEIQRTEQGDSAMYLCASSSTGGHNEQFFGPGTRLTVL

SEQ ID NO: 97 - protein, 113 aa, Artificial Sequence
  Synthetic sequence TCR1,13 alpha chain variable region (mature)
QQGEEDPQALSIQEGENATMNCSYKTSINNLQWYRQNSGRGLVHLILIRSNEREKHSGRLRVTLDTSKKSSSLLITASRAADTASYFCATKRDSGAGSYQLTFGKGTKLSVIP

SEQ ID NO: 98 - protein, 110 aa, Artificial Sequence
  Synthetic sequence TCR2,14 beta chain variable region (mature)
GVSQDPRHKITKRGQNVTFRCDPISEHNRLYWYRQTLGQGPEFLTYFQNEAQLEKSRLLSDRFSAERPKGSFSTLEIQRTEQGDSAMYLCASSLVKGEKLFGSGTQLSVL

SEQ ID NO: 99 - protein, 112 aa, Artificial Sequence
  Synthetic sequence TCR2,14 alpha chain variable region (mature)
KQEVTQIPAALSVPEGENLVLNCSFTDSAIYNLQWFRQDPGKGLTSLLLIQSSQREQTSGRLNASDKSSGRSTLYIAASQPGDSATYLCAVIGLGGTYKYIFGTGTRLKVLA

SEQ ID NO: 100 - protein, 111 aa, Artificial Sequence
  Synthetic sequence TCR5 beta chain variable region (mature)
GVSQDPRHKITKRGQNVTFRCDPISEHNRLYWYRQTLGQGPEFLTYFQNEAQLEKSRLLSDRFSAERPKGSFSTLEIQRTEQGDSAMYLCASSLTTLDEQYVGPGTRLTVT

SEQ ID NO: 101 - protein, 109 aa, Artificial Sequence
  Synthetic sequence TCR5 alpha chain variable region (mature)
QQGEEDPQALSIQEGENATMNCSYKTSINNLQWYRQNSGRGLVHLILIRSNEREKHSGRLRVTLDTSKKSSSLLITASRAADTASYFCATNSGNTPLVFGKGTRLSVIA

SEQ ID NO: 102 - protein, 111 aa, Artificial Sequence
  Synthetic sequence TCR10 beta chain variable region (mature)
GVSQDPRHKITKRGQNVTFRCDPISEHNRLYWYRQTLGQGPEFLTYFQNEAQLEKSRLLSDRFSAERPKGSFSTLEIQRTEQGDSAMYLCASSMLTNYEQYFGPGTRLTVT

SEQ ID NO: 103 - protein, 113 aa, Artificial Sequence
  Synthetic sequence TCR10 alpha chain variable region (mature)
KNQVEQSPQSLIILEGKNCTLQCNYTVSPFSNLRWYKQDTGRGPVSLTIMTFSENTKSNGRYTATLDADTKQSSLHITASQLSDSASYICVVDSGGGADGLTFGKGTHLIIQP

SEQ ID NO: 104 - protein, 111 aa, Artificial Sequence
  Synthetic sequence TCR16 beta chain variable region (mature)
GVSQDPRHKITKRGQNVTFRCDPISEHNRLYWYRQTLGQGPEFLTYFQNEAQLEKSRLLSDRFSAERPKGSFSTLEIQRTEQGDSAMYLCASSLVVGNEQFFGPGTRLTVL

SEQ ID NO: 105 - protein, 112 aa, Artificial Sequence
  Synthetic sequence TCR16 alpha chain variable region (mature)
KQEVTQIPAALSVPEGENLVLNCSFTDSAIYNLQWFRQDPGKGLTSLLLIQSSQREQTSGRLNASLDKSSGRSTLYIAASQPGDSATYLCAVHLLNDYKLSFGAGTTVTVRA

SEQ ID NO: 106 - protein, 111 aa, Artificial Sequence
  Synthetic sequence TCR29 beta chain variable region (mature)
GVSQDPRHKITKRGQNVTFRCDPISEHNRLYWYRQTLGQGPEFLTYFQNEAQLEKSRLLSDRFSAERPKGSFSTLEIQRTEQGDSAMYLCASSLVSGNTIYFGEGSWLTVV

SEQ ID NO: 107 - protein, 115 aa, Artificial Sequence
  Synthetic sequence TCR29 alpha chain variable region (mature)
KQEVTQIPAALSVPEGENLVLNCSFTDSAIYNLQWFRQDPGKGLTSLLLIQSSQREQTSGRLNASLDKSSGRSTLYIAASQPGDSATYLCAVRGGTTSGTYKYIFGTGTRLKVLA

SEQ ID NO: 108 - protein, 289 aa, Artificial Sequence
  Synthetic sequence TCR1,13 beta chain (full length) (Cys modified) (mature)
GVSQDPRHKITKRGQNVTFRCDPISEHNRLYWYRQTLGQGPEFLTYFQNEAQLEKSRLLSDRFSAERPKGSFSTLEIQRTEQGDSAMYLCASSSTGGHNEQFFGPGTRLTVLEDLKNVFPPEVAVFEPSEAEISHTQKATLVCLATGFYPDHVELSWWVNGKEVHSGVCTDPQPLKEQPALNDSRYCLSSRLRVSATFWQNPRNHFRCQVQFYGLSENDEWTQDRAKPVTQIVSAEAWGRADCGFTSESYQQGVLSATILYEILLGKATLYAVLVSALVLMAMVKRKDS

SEQ ID NO: 109 - protein, 254 aa, Artificial Sequence
  Synthetic sequence TCR1,13 alpha chain (full length)(Cys modified) (mature)
QQGEEDPQALSIQEGENATMNCSYKTSINNLQWYRQNSGRGLVHLILIRSNEREKHSGRLRVTLDTSKKSSSLLITASRAADTASYFCATKRDSGAGSYQLTFGKGTKLSVIPNIQNPDPAVYQLRDSKSSDKSVCLFTDFDSQTNVSQSKDSDVYITDKCVLDMRSMDFKSNSAVAWSNKSDFACANAFNNSIIPEDTFFPSPESSCDVKLVEKSFETDTNLNFQNLSVIGFRILLLKVAGFNLLMTLRLWSS

SEQ ID NO: 110 - protein, 287 aa, Artificial Sequence
  Synthetic sequence TCR2,14 beta chain (full length) (Cys modified) (mature)
GVSQDPRHKITKRGQNVTFRCDPISEHNRLYWYRQTLGQGPEFLTYFQNEAQLEKSRLLSDRFSAERPKGSFSTLEIQRTEQGDSAMYLCASSLVKGEKLFFGSGTQLSVLEDLNKVFPPEVAVFEPSEAEISHTQKATLVCLATGFFPDHVELSWWVNGKEVHSGVCTDPQPLKEQPALNDSRYCLSSRLRVSATFWQNPRNHFRCQVQFYGLSENDEWTQDRAKPVTQIVSAEAWGRADCGFTSVSYQQGVLSATILYEILLGKATLYAVLVSALVLMAMVKRKD

SEQ ID NO: 111 - protein, 254 aa, Artificial Sequence
  Synthetic sequence TCR2,14 alpha chain (full length)(Cys modified) (mature)
KQEVTQIPAALSVPEGENLVLNCSFTDSAIYNLQWFRQDPGKGLTSLLLIQSSQREQTSGRLNASLDKSSGRSTLYIAASQPGDSATYLCAVIGLGGTYKYIFGTGTRLKVLANIQNPDPAVYQLRDSKSSDKSVCLFTDFDSQTNVSQSKDSDVYITDKCVLDMRSMDFKSNSAVAWSNKSDFACANAFNNSIIPEDTFFPSPESSCDVKLVEKSFETDTNLNFQNLSVIGFRILLLKVAGFNLLMTLRLWSS

SEQ ID NO: 112 - protein, 288 aa, Artificial Sequence
  Synthetic sequence TCR5 beta chain (full length) (Cys modified) (mature)
GVSQDPRHKITKRGQNVTFRCDPISEHNRLYWYRQTLGQGPEFLTYFQNEAQLEKSRLLSDRFSAERPKGSFSTLEIQRTEQGDSAMYLCASSLTTLDEQYVGPGTRLTVTEDLKNVFPPEVAVFEPSEAEISHTQKATLVCLATGFYPDHVELSWWVNGKEVHSGVCTDPQPLKEQPALNDSRYCLSSRLRVSATFWQNPRNHFRCQVQFYGLSENDEWTQDRAKPVTQIVSAEAWGRADCGFTSESYQQGVLSATILYEILLGKATLYAVLVSALVLMAMVKRKDS

SEQ ID NO: 113 - protein, 250 aa, Artificial Sequence
  Synthetic sequence TCR5 alpha chain (full length)(Cys modified) (mature)
QQGEEDPQALSIQEGENATMNCSYKTSINNLQWYRQNSGRGLVHLILIRSNEREKHSGRLRVTLDTSKKSSSLLITASRAADTASYFCATNSGNTPLVFGKGTRLSVIANIQNPDPAVYQLRDSKSSDKSVCLFTDFDSQTNVSQSKDSDVYITDKCVLDMRSMDFKSNSAVAWSNKSDFACANAFNNSIIPEDTFFPSPESSCDVKLVEKSFETDTNLNFQNLSVIGFRILLLKVAGFNLLMTLRLWSS

SEQ ID NO: 114 - protein, 288 aa, Artificial Sequence
  Synthetic sequence TCR10 beta chain (full length) (Cys modified) (mature)
GVSQDPRHKITKRGQNVTFRCDPISEHNRLYWYRQTLGQGPEFLTYFQNEAQLEKSRLLSDRFSAERPKGSFSTLEIQRTEQGDSAMYLCASSMLTNYEQYFGPGTRLTVTEDLKNVFPPEVAVFEPSEAEISHTQKATLVCLATGFYPDHVELSWWVNGKEVHSGVCTDPQPLKEQPALNDSRYCLSSRLRVSATFWQNPRNHFRCQVQFYGLSENDEWTQDRAKPVTQIVSAEAWGRADCGFTSESYQQGVLSATILYEILLGKATLYAVLVSALVLMAMVKRKDS

SEQ ID NO: 115 - protein, 254 aa, Artificial Sequence
  Synthetic sequence TCR10 alpha chain (full length)(Cys modified) (mature)
KNQVEQSPQSLIILEGKNCTLQCNYTVSPFSNLRWYKQDTGRGPVSLTIMTFSENTKSNGRYTATLDADTKQSSLHITASQLSDSASYICVVDSGGGADGLTFGKGTHLIIQPYIQNPDPAVYQLRDSKSSDKSVCLFTDFDSQTNVSQSKDSDVYITDKCVLDMRSMDFKSNSAVAWSNKSDFACANAFNNSIIPEDTFFPSPESSCDVKLVEKSFETDTNLNFQNLSVIGFRILLLKVAGFNLLMTLRLWSS

SEQ ID NO: 116 - protein, 287 aa, Artificial Sequence
  Synthetic sequence TCR16 beta chain (full length) (Cys modified) (mature)
GVSQDPRHKITKRGQNVTFRCDPISEHNRLYWYRQTLGQGPEFLTYFQNEAQLEKSRLLSDRFSAERPKGSFSTLEIQRTEQGDSAMYLCASSLVVGNEQFFGPGTRLTVLEDLKNVFPPEVAVFEPSEAEISHTQKATLVCLATGFYPDHVELSWWVNGKEVHSGVCTDPQPLKEQPALNDSRYCLSSRLRVSATFWQNPRNHFRCQVQFYGLSENDEWTQDRAKPVTQIVSAEAWGRADCGFTSESYQQGVLSATILYEILLGKATLYAVLVSALVLMAMVKRKD

SEQ ID NO: 117 - protein, 253 aa, Artificial Sequence
  Synthetic sequence TCR16 alpha chain (full length) (Cys modified) (mature)
KQEVTQIPAALSVPEGENLVLNCSFTDSAIYNLQWFRQDPGKGLTSLLLIQSSQREQTSGRLNASLDKSSGRSTLYIAASQPGDSATYLCAVHLLNDYKLSFGAGTTVTVRANIQNPDPAVYQLRDSKSSDKSVCLFTDFDSQTNVSQSKDSDVYITDKCVLDMRSMDFKSNSAVAWSNKSDFACANAFNNSIIPEDTFFPSPESSCDVKLVEKSFETDTNLNFQNLSVIGFRILLLKVAGFNLLMTLRLWSS

SEQ ID NO: 118 - protein, 288 aa, Artificial Sequence
  Synthetic sequenceTCR29 beta chain (full length) (mature)
GVSQDPRHKITKRGQNVTFRCDPISEHNRLYWYRQTLGQGPEFLTYFQNEAQLEKSRLLSDRFSAERPKGSFSTLEIQRTEQGDSAMYLCASSLVSGNTIYFGEGSWLTVVEDLNKVFPPEVAVFEPSEAEISHTQKATLVCLATGFFPDHVELSWWVNGKEVHSGVSTDPQPLKEQPALNDSRYCLSSRLRVSATFWQNPRNHFRCQVQFYGLSENDEWTQDRAKPVTQIVSAEAWGRADCGFTSVSYQQGVLSATILYEILLGKATLYAVLVSALVLMAMVKRKDF

SEQ ID NO: 119 - protein, 256 aa, Artificial Sequence
  Synthetic sequence TCR29 alpha chain (full length) (mature)
KQEVTQIPAALSVPEGENLVLNCSFTDSAIYNLQWFRQDPGKGLTSLLLIQSSQREQTSGRLNASLDKSSGRSTLYIAASQPGDSATYLCAVRGGTTSGTYKYIFGTGTRLKVLANIQNPDPAVYQLRDSKSSDKSVCLFTDFDSQTNVSQSKDSDVYITDKTVLDMRSMDFKSNSAVAWSNKSDFACANAFNNSIIPEDTFFPSPESSCDVKLVEKSFETDTNLNFQNLSVIGFRILLLKVAGFNLLMTLRLWSS

SEQ ID NO: 120 - protein, 214 aa, Artificial Sequence
  Synthetic sequence CD8 co-receptor alpha chain (mature)
SQFRVSPLDRTWNLGETVELKCQVLLSNPTSGCSWLFQPRGAAASPTFLLYLSQNKPKAAEGLDTQRFSGKRLGDTFVLTLSDFRRENEGYYFCSALSNSIMYFSHFVPVFLPAKPTTTPAPRPPTPAPTIASQPLSLRPEACRPAAGGAVHTRGLDFACDIYIWAPLAGTCGVLLLSLVITLYCNHRNRRRVCKCPRPVVKSGDKPSLSARYV

SEQ ID NO: 121 - protein, 189 aa, Artificial Sequence
  Synthetic sequence CD8 co-receptor beta chain isoform 1 (mature)
LQQTPAYIKVQTNKMVMLSCEAKISLSNMRIYWLRQRQAPSSDSHHEFLALWDSAKGTIHGEEVEQEKIAVFRDASRFILNLTSVKPEDSGIYFCMIVGSPELTFGKGTQLSVVDFLPTTAQPTKKSTLKKRVCRLPRPETQKGPLCSPITLGLLVAGVLVLLVSLGVAIHLCCRRRRARLRFMKQFYK

SEQ ID NO: 122 - protein, 200 aa, Artificial Sequence
  Synthetic sequence CD8 co-receptor beta chain isoform 2 (mature)
LQQTPAYIKVQTNKMVMLSCEAKISLSNMRIYWLRQRQAPSSDSHHEFLALWDSAKGTIHGEEVEQEKIAVFRDASRFILNLTSVKPEDSGIYFCMIVGSPELTFGKGTQLSVVDFLPTTAQPTKKSTLKKRVCRLPRPETQKGPLCSPITLGLLVAGVLVLLVSLGVAIHLCCRRRRARLRFMKQLRLHPLEKCSRMDY

SEQ ID NO: 123 - protein, 225 aa, Artificial Sequence
  Synthetic sequence CD8 co-receptor beta chain isoform 3 (mature)
LQQTPAYIKVQTNKMVMLSCEAKISLSNMRIYWLRQRQAPSSDSHHEFLALWDSAKGTIHGEEVEQEKIAVFRDASRFILNLTSVKPEDSGIYFCMIVGSPELTFGKGTQLSVVDFLPTTAQPTKKSTLKKRVCRLPRPETQKGPLCSPITLGLLVAGVLVLLVSLGVAIHLCCRRRRARLRFMKQKFNIVCLKISGFTTCCCFQILQISREYGFGVLLQKDIGQ

SEQ ID NO: 124 - protein, 225 aa, qArtificial Sequence; identical to SEQ ID NO: 123
  Synthetic sequence CD8 co-receptor beta chain isoform 4 (mature)

SEQ ID NO: 125 - protein, 222 aa, Artificial Sequence
  Synthetic sequence CD8 co-receptor beta chain isoform 5 (mature)
LQQTPAYIKVQTNKMVMLSCEAKISLSNMRIYWLRQRQAPSSDSHHEFLALWDSAKGTIHGEEVEQEKIAVFRDASRFILNLTSVKPEDSGIYFCMIVGSPELTFGKGTQLSVVDFLPTTAQPTKKSTLKKRVCRLPRPETQKGPLCSPITLGLLVAGVLVLLVSLGVAIHLCCRRRRARLRFMKQPQGEGISGTFVPQCLHGYYSNTTTSQKLLNPWILKT

SEQ ID NO: 126 - DNA, 930 bp, Artificial Sequence
  Synthetic sequence TCR 29 beta chain (wild-type)
atgggcaccagcctcctctgctggatggccctgtgtctcctgggggcagatcacgcagatactggagtctcccaggaccccagacacaagatcacaaagaggggacagaatgtaactttcaggtgtgatccaatttctgaacacaaccgcctttattggtaccgacagaccctggggcagggcccagagtttctgacttacttccagaatgaagctcaactagaaaaatcaaggctgctcagtgatcggttctctgcagagaggcctaagggatctttctccaccttggagatccagcgcacagagcagggggactcggccatgtatctctgtgccagcagcttagtatccggaaacaccatatattttggagagggaagttggctcactgttgtagaggacctgaacaaggtgttcccacccgaggtcgctgtgtttgagccatcagaagcagagatctcccacacccaaaaggccacactggtgtgcctggccacaggcttcttccccgaccacgtggagctgagctggtgggtgaatgggaaggaggtgcacagtggggtcagcacagacccgcagcccctcaaggagcagcccgccctcaatgactccagatactgcctgagcagccgcctgagggtctcggccaccttctggcagaacccccgcaaccacttccgctgtcaagtccagttctacgggctctcggagaatgacgagtggacccaggatagggccaaacccgtcacccagatcgtcagcgccgaggcctggggtagagcagactgtggctttacctcggtgtcctaccagcaaggggtcctgtctgccaccatcctctatgagatcctgctagggaaggccaccctgtatgctgtgctggtcagcgcccttgtgttgatggccatggtcaagagaaaggatttctga

SEQ ID NO: 127 - DNA, 828 bp, Artificial Sequence
  Synthetic sequence TCR 29 alpha chain (wild-type)
atggagaccctcttgggcctgcttatcctttggctgcagctgcaatgggtgagcagcaaacaggaggtgacgcagattcctgcagctctgagtgtcccagaaggagaaaacttggttctcaactgcagtttcactgatagcgctatttacaacctccagtggtttaggcaggaccctgggaaaggtctcacatctctgttgcttattcagtcaagtcagagagagcaaacaagtggaagacttaatgcctcgctggataaatcatcaggacgtagtactttatacattgcagcttctcagcctggtgactcagccacctacctctgtgctgtgagaggggggactacctcaggaacctacaaatacatctttggaacaggcaccaggctgaaggttttagcaaatatccagaaccctgaccctgccgtgtaccagctgagagactctaaatccagtgacaagtctgtctgcctattcaccgattttgattctcaaacaaatgtgtcacaaagtaaggattctgatgtgtatatcacagacaaaactgtgctagacatgaggtctatggacttcaagagcaacagtgctgtggcctggagcaacaaatctgactttgcatgtgcaaacgccttcaacaacagcattattccagaagacaccttcttccccagcccagaaagttcctgtgatgtcaagctggtcgagaaaagctttgaaacagatacgaacctaaactttcaaaacctgtcagtgattgggttccgaatcctcctcctgaaagtggccgggtttaatctgctcatgacgctgcggctgtggtccagctga